European Patent Application EP 4 512 428 A2, published February 26, 2025. Title: METHODS OF USING BISPECIFIC ANTIGEN-BINDING CONSTRUCTS TARGETING HER2. Applicant: ZYMEWORKS BC INC. Application undefined NOT YET ASSIGNED, filed November 26, 2015. The sequence listing filed with the application follows.

SEQUENCE LISTING (350 sequences)

SEQ ID NO: 1 - protein, 450 aa, synthetic construct
  REGION 1..450: note = Description of Artificial Sequence: Synthetic polypeptide
EVQLVESGGGLVQPGGSLRLSCAASGFNIKDTYIHWVRQAPGKGLEWVARIYPTNGYTRYADSVKGRFTISADTSKNTAYLQMNSLRAEDTAVYYCSRWGGDGFYAMDYWGQGTLVTVSSASTKGPSVFPLAPSSKSTSGGTAALGCLVKDYFPEPVTVSWNSGALTSGVHTFPAVLQSSGLYSLSSVVTVPSSSLGTQTYICNVNHKPSNTKVDKKVEPKSCDKTHTCPPCPAPELLGGPSVFLFPPKPKDTLMISRTPEVTCVVVDVSHEDPEVKFNWYVDGVEVHNAKTKPREEQYNSTYRVVSVLTVLHQDWLNGKEYKCKVSNKALPAPIEKTISKAKGQPREPQVYTLPPSRDELTKNQVSLTCLVKGFYPSDIAVEWESNGQPENNYKTTPPVLDSDGSFFLYSKLTVDKSRWQQGNVFSCSVMHEALHNHYTQKSLSLSPGK

SEQ ID NO: 2 - DNA, 1350 bp, synthetic construct
  misc_feature 1..1350: note = Description of Artificial Sequence: Synthetic polynucleotide
  source 1..1350: mol_type = other DNA
gaggtgcagctggtggaaagcggaggaggactggtgcagccaggaggatctctgcgactgagttgcgccgcttcaggattcaacatcaaggacacctacattcactgggtgcgacaggctccaggaaaaggactggagtgggtggctcgaatctatcccactaatggatacacccggtatgccgactccgtgaaggggaggtttactattagcgccgatacatccaaaaacactgcttacctgcagatgaacagcctgcgagccgaagataccgctgtgtactattgcagtcgatggggaggagacggattctacgctatggattattggggacaggggaccctggtgacagtgagctccgcctctaccaagggccccagtgtgtttcccctggctccttctagtaaatccacctctggagggacagccgctctgggatgtctggtgaaggactatttccccgagcctgtgaccgtgagttggaactcaggcgccctgacaagcggagtgcacacttttcctgctgtgctgcagtcaagcgggctgtactccctgtcctctgtggtgacagtgccaagttcaagcctgggcacacagacttatatctgcaacgtgaatcataagccctcaaatacaaaagtggacaagaaagtggagcccaagagctgtgataagacccacacctgccctccctgtccagctccagaactgctgggaggacctagcgtgttcctgtttccccctaagccaaaagacactctgatgatttccaggactcccgaggtgacctgcgtggtggtggacgtgtctcacgaggaccccgaagtgaagttcaactggtacgtggatggcgtggaagtgcataatgctaagacaaaaccaagagaggaacagtacaactccacttatcgcgtcgtgagcgtgctgaccgtgctgcaccaggactggctgaacgggaaggagtataagtgcaaagtcagtaataaggccctgcctgctccaatcgaaaaaaccatctctaaggccaaaggccagccaagggagccccaggtgtacacactgccacccagcagagacgaactgaccaagaaccaggtgtccctgacatgtctggtgaaaggcttctatcctagtgatattgctgtggagtgggaatcaaatggacagccagagaacaattacaagaccacacctccagtgctggacagcgatggcagcttcttcctgtattccaagctgacagtggataaatctcgatggcagcaggggaacgtgtttagttgttcagtgatgcatgaagccctgcacaatcattacactcagaagagcctgtccctgtctcccggcaaa

SEQ ID NO: 3 - protein, 120 aa, synthetic construct [sequence omitted]

SEQ ID NO: 4 - DNA, 360 bp, synthetic construct
  misc_feature 1..360: note = Description of Artificial Sequence: Synthetic polynucleotide
  source 1..360: mol_type = other DNA
gaggtgcagctggtggaaagcggaggaggactggtgcagccaggaggatctctgcgactgagttgcgccgcttcaggattcaacatcaaggacacctacattcactgggtgcgacaggctccaggaaaaggactggagtgggtggctcgaatctatcccactaatggatacacccggtatgccgactccgtgaaggggaggtttactattagcgccgatacatccaaaaacactgcttacctgcagatgaacagcctgcgagccgaagataccgctgtgtactattgcagtcgatggggaggagacggattctacgctatggattattggggacaggggaccctggtgacagtgagctcc

SEQ ID NO: 5 - protein, 8 aa, synthetic construct
  REGION 1..8: note = Description of Artificial Sequence: Synthetic peptide
GFNIKDTY

SEQ ID NO: 6 - DNA, 24 bp, synthetic construct
  misc_feature 1..24: note = Description of Artificial Sequence: Synthetic oligonucleotide
  source 1..24: mol_type = other DNA
ggattcaacatcaaggacacctac

SEQ ID NO: 7 - protein, 13 aa, synthetic construct
  REGION 1..13: note = Description of Artificial Sequence: Synthetic peptide
SRWGGDGFYAMDY

SEQ ID NO: 8 - DNA, 39 bp, synthetic construct
  misc_feature 1..39: note = Description of Artificial Sequence: Synthetic oligonucleotide
  source 1..39: mol_type = other DNA
agtcgatggggaggagacggattctacgctatggattat

SEQ ID NO: 9 - protein, 8 aa, synthetic construct
  REGION 1..8: note = Description of Artificial Sequence: Synthetic peptide
IYPTNGYT

SEQ ID NO: 10 - DNA, 24 bp, synthetic construct
  misc_feature 1..24: note = Description of Artificial Sequence: Synthetic oligonucleotide
  source 1..24: mol_type = other DNA
atctatcccactaatggatacacc

SEQ ID NO: 11 - protein, 98 aa, synthetic construct
  REGION 1..98: note = Description of Artificial Sequence: Synthetic polypeptide
ASTKGPSVFPLAPSSKSTSGGTAALGCLVKDYFPEPVTVSWNSGALTSGVHTFPAVLQSSGLYSLSSVVTVPSSSLGTQTYICNVNHKPSNTKVDKKV

SEQ ID NO: 12 - DNA, 294 bp, synthetic construct
  misc_feature 1..294: note = Description of Artificial Sequence: Synthetic polynucleotide
  source 1..294: mol_type = other DNA
gcctctaccaagggccccagtgtgtttcccctggctccttctagtaaatccacctctggagggacagccgctctgggatgtctggtgaaggactatttccccgagcctgtgaccgtgagttggaactcaggcgccctgacaagcggagtgcacacttttcctgctgtgctgcagtcaagcgggctgtactccctgtcctctgtggtgacagtgccaagttcaagcctgggcacacagacttatatctgcaacgtgaatcataagccctcaaatacaaaagtggacaagaaagtg

SEQ ID NO: 13 - protein, 110 aa, synthetic construct
  REGION 1..110: note = Description of Artificial Sequence: Synthetic polypeptide
APELLGGPSVFLFPPKPKDTLMISRTPEVTCVVVDVSHEDPEVKFNWYVDGVEVHNAKTKPREEQYNSTYRVVSVLTVLHQDWLNGKEYKCKVSNKALPAPIEKTISKAK

SEQ ID NO: 14 - DNA, 330 bp, synthetic construct
  misc_feature 1..330: note = Description of Artificial Sequence: Synthetic polynucleotide
  source 1..330: mol_type = other DNA
gctccagaactgctgggaggacctagcgtgttcctgtttccccctaagccaaaagacactctgatgatttccaggactcccgaggtgacctgcgtggtggtggacgtgtctcacgaggaccccgaagtgaagttcaactggtacgtggatggcgtggaagtgcataatgctaagacaaaaccaagagaggaacagtacaactccacttatcgcgtcgtgagcgtgctgaccgtgctgcaccaggactggctgaacgggaaggagtataagtgcaaagtcagtaataaggccctgcctgctccaatcgaaaaaaccatctctaaggccaaa

SEQ ID NO: 15 - protein, 106 aa, synthetic construct [sequence omitted]

SEQ ID NO: 16 - DNA, 318 bp, synthetic construct
  misc_feature 1..318: note = Description of Artificial Sequence: Synthetic polynucleotide
  source 1..318: mol_type = other DNA
ggccagccaagggagccccaggtgtacacactgccacccagcagagacgaactgaccaagaaccaggtgtccctgacatgtctggtgaaaggcttctatcctagtgatattgctgtggagtgggaatcaaatggacagccagagaacaattacaagaccacacctccagtgctggacagcgatggcagcttcttcctgtattccaagctgacagtggataaatctcgatggcagcaggggaacgtgtttagttgttcagtgatgcatgaagccctgcacaatcattacactcagaagagcctgtccctgtctcccggc

SEQ ID NO: 17 - protein, 448 aa, synthetic construct
  REGION 1..448: note = Description of Artificial Sequence: Synthetic polypeptide
EVQLVESGGGLVQPGGSLRLSCAASGFTFTDYTMDWVRQAPGKGLEWVADVNPNSGGSIYNQRFKGRFTLSVDRSKNTLYLQMNSLRAEDTAVYYCARNLGPSFYFDYWGQGTLVTVSSASTKGPSVFPLAPSSKSTSGGTAALGCLVKGYFPEPVTVSWNSGALTSGVHTFPAVLKSSGLYSLSSVVTVPSSSLGTQTYICNVNHKPSNTKVDKKVEPKSCDKTHTCPPCPAPELLGGPSVFLFPPKPKDTLMISRTPEVTCVVVDVSHEDPEVKFNWYVDGVEVHNAKTKPREEQYNSTYRVVSVLTVLHQDWLNGKEYKCKVSNKALPAPIEKTISKAKGQPREPQVYVLPPSRDELTKNQVSLLCLVKGFYPSDIAVEWESNGQPENNYLTWPPVLDSDGSFFLYSKLTVDKSRWQQGNVFSCSVMHEALHNHYTQKSLSLSPG

SEQ ID NO: 18 - DNA, 1344 bp, synthetic construct
  misc_feature 1..1344: note = Description of Artificial Sequence: Synthetic polynucleotide
  source 1..1344: mol_type = other DNA
gaagtgcagctggtcgaatctggaggaggactggtgcagccaggagggtccctgcgcctgtcttgcgccgctagtggcttcacttttaccgactacaccatggattgggtgcgacaggcacctggaaagggcctggagtgggtcgccgatgtgaacccaaatagcggaggctccatctacaaccagcggttcaagggccggttcaccctgtcagtggaccggagcaaaaacaccctgtatctgcagatgaatagcctgcgagccgaagatactgctgtgtactattgcgcccggaatctggggccctccttctactttgactattgggggcagggaactctggtcaccgtgagctccgcctccaccaagggaccttctgtgttcccactggctccctctagtaaatccacatctgggggaactgcagccctgggctgtctggtgaagggctacttcccagagcccgtcacagtgtcttggaacagtggcgctctgacttctggggtccacacctttcctgcagtgctgaagtcaagcgggctgtacagcctgtcctctgtggtcaccgtgccaagttcaagcctgggaacacagacttatatctgcaacgtgaatcacaagccatccaatacaaaagtcgacaagaaagtggaacccaagtcttgtgataaaacccatacatgccccccttgtcctgcaccagagctgctgggaggaccaagcgtgttcctgtttccacccaagcctaaagatacactgatgattagtaggaccccagaagtcacatgcgtggtcgtggacgtgagccacgaggaccccgaagtcaagtttaactggtacgtggacggcgtcgaggtgcataatgccaagactaaacccagggaggaacagtacaacagtacctatcgcgtcgtgtcagtcctgacagtgctgcatcaggattggctgaacgggaaagagtataagtgcaaagtgagcaataaggctctgcccgcacctatcgagaaaacaatttccaaggcaaaaggacagcctagagaaccacaggtgtacgtgctgcctccatcaagggatgagctgacaaagaaccaggtcagcctgctgtgtctggtgaaaggattctatccctctgacattgctgtggagtgggaaagtaatggccagcctgagaacaattacctgacctggccccctgtgctggactcagatggcagcttctttctgtatagcaagctgaccgtcgacaaatcccggtggcagcaggggaatgtgtttagttgttcagtcatgcacgaggcactgcacaaccattacacccagaagtcactgtcactgtcaccaggg

SEQ ID NO: 19 - protein, 119 aa, synthetic construct [sequence omitted]

SEQ ID NO: 20 - DNA, 357 bp, synthetic construct
  misc_feature 1..357: note = Description of Artificial Sequence: Synthetic polynucleotide
  source 1..357: mol_type = other DNA
gaagtgcagctggtcgaatctggaggaggactggtgcagccaggagggtccctgcgcctgtcttgcgccgctagtggcttcacttttaccgactacaccatggattgggtgcgacaggcacctggaaagggcctggagtgggtcgccgatgtgaacccaaatagcggaggctccatctacaaccagcggttcaagggccggttcaccctgtcagtggaccggagcaaaaacaccctgtatctgcagatgaatagcctgcgagccgaagatactgctgtgtactattgcgcccggaatctggggccctccttctactttgactattgggggcagggaactctggtcaccgtgagctcc

SEQ ID NO: 21 - protein, 8 aa, synthetic construct
  REGION 1..8: note = Description of Artificial Sequence: Synthetic peptide
GFTFTDYT

SEQ ID NO: 22 - DNA, 24 bp, synthetic construct
  misc_feature 1..24: note = Description of Artificial Sequence: Synthetic oligonucleotide
  source 1..24: mol_type = other DNA
ggcttcacttttaccgactacacc

SEQ ID NO: 23 - protein, 12 aa, synthetic construct
  REGION 1..12: note = Description of Artificial Sequence: Synthetic peptide
ARNLGPSFYFDY

SEQ ID NO: 24 - DNA, 36 bp, synthetic construct
  misc_feature 1..36: note = Description of Artificial Sequence: Synthetic oligonucleotide
  source 1..36: mol_type = other DNA
gcccggaatctggggccctccttctactttgactat

SEQ ID NO: 25 - protein, 8 aa, synthetic construct
  REGION 1..8: note = Description of Artificial Sequence: Synthetic peptide
VNPNSGGS

SEQ ID NO: 26 - DNA, 24 bp, synthetic construct
  misc_feature 1..24: note = Description of Artificial Sequence: Synthetic oligonucleotide
  source 1..24: mol_type = other DNA
gtgaacccaaatagcggaggctcc

SEQ ID NO: 27 - protein, 98 aa, synthetic construct
  REGION 1..98: note = Description of Artificial Sequence: Synthetic polypeptide
ASTKGPSVFPLAPSSKSTSGGTAALGCLVKGYFPEPVTVSWNSGALTSGVHTFPAVLKSSGLYSLSSVVTVPSSSLGTQTYICNVNHKPSNTKVDKKV

SEQ ID NO: 28 - DNA, 294 bp, synthetic construct
  misc_feature 1..294: note = Description of Artificial Sequence: Synthetic polynucleotide
  source 1..294: mol_type = other DNA
gcctccaccaagggaccttctgtgttcccactggctccctctagtaaatccacatctgggggaactgcagccctgggctgtctggtgaagggctacttcccagagcccgtcacagtgtcttggaacagtggcgctctgacttctggggtccacacctttcctgcagtgctgaagtcaagcgggctgtacagcctgtcctctgtggtcaccgtgccaagttcaagcctgggaacacagacttatatctgcaacgtgaatcacaagccatccaatacaaaagtcgacaagaaagtg

SEQ ID NO: 29 - protein, 110 aa, synthetic construct; identical to SEQ ID NO: 13
  REGION 1..110: note = Description of Artificial Sequence: Synthetic polypeptide

SEQ ID NO: 30 - DNA, 330 bp, synthetic construct
  misc_feature 1..330: note = Description of Artificial Sequence: Synthetic polynucleotide
  source 1..330: mol_type = other DNA
gcaccagagctgctgggaggaccaagcgtgttcctgtttccacccaagcctaaagatacactgatgattagtaggaccccagaagtcacatgcgtggtcgtggacgtgagccacgaggaccccgaagtcaagtttaactggtacgtggacggcgtcgaggtgcataatgccaagactaaacccagggaggaacagtacaacagtacctatcgcgtcgtgtcagtcctgacagtgctgcatcaggattggctgaacgggaaagagtataagtgcaaagtgagcaataaggctctgcccgcacctatcgagaaaacaatttccaaggcaaaa

SEQ ID NO: 31 - protein, 106 aa, synthetic construct
  REGION 1..106: note = Description of Artificial Sequence: Synthetic polypeptide
GQPREPQVYVLPPSRDELTKNQVSLLCLVKGFYPSDIAVEWESNGQPENNYLTWPPVLDSDGSFFLYSKLTVDKSRWQQGNVFSCSVMHEALHNHYTQKSLSLSPG

SEQ ID NO: 32 - DNA, 318 bp, synthetic construct
  misc_feature 1..318: note = Description of Artificial Sequence: Synthetic polynucleotide
  source 1..318: mol_type = other DNA
ggacagcctagagaaccacaggtgtacgtgctgcctccatcaagggatgagctgacaaagaaccaggtcagcctgctgtgtctggtgaaaggattctatccctctgacattgctgtggagtgggaaagtaatggccagcctgagaacaattacctgacctggccccctgtgctggactcagatggcagcttctttctgtatagcaagctgaccgtcgacaaatcccggtggcagcaggggaatgtgtttagttgttcagtcatgcacgaggcactgcacaaccattacacccagaagtcactgtcactgtcaccaggg

SEQ ID NO: 33 - protein, 214 aa, synthetic construct
  REGION 1..214: note = Description of Artificial Sequence: Synthetic polypeptide
DIQMTQSPSSLSASVGDRVTITCKASQDVSIGVAWYQQKPGKAPKLLIYSASYRYTGVPSRFSGSGSGTDFTLTISSLQPEDFATYYCQQYYIYPYTFGQGTKVEIKRTVAAPSVFIFPPSDEQLKSGTASVVCLLNNFYPREAKVQWKVDNALQSGNSQESVTEQDSKDSTYSLSSTLTLSKADYEKHKVYACEVTHQGLSSPVTKSFNRGEC

SEQ ID NO: 34 - DNA, 642 bp, synthetic construct
  misc_feature 1..642: note = Description of Artificial Sequence: Synthetic polynucleotide
  source 1..642: mol_type = other DNA
gatattcagatgacccagtccccaagctccctgagtgcctcagtgggcgaccgagtcaccatcacatgcaaggcttcccaggatgtgtctattggagtcgcatggtaccagcagaagccaggcaaagcacccaagctgctgatctatagcgcctcctaccggtataccggcgtgccctctagattctctggcagtgggtcaggaacagactttactctgaccatctctagtctgcagcctgaggatttcgctacctactattgccagcagtactatatctacccatatacctttggccaggggacaaaagtggagatcaagaggactgtggccgctccctccgtcttcatttttcccccttctgacgaacagctgaaaagtggcacagccagcgtggtctgtctgctgaacaatttctaccctcgcgaagccaaagtgcagtggaaggtcgataacgctctgcagagcggcaacagccaggagtctgtgactgaacaggacagtaaagattcaacctatagcctgtcaagcacactgactctgagcaaggcagactacgagaagcacaaagtgtatgcctgcgaagtcacacatcaggggctgtcctctcctgtgactaagagctttaacagaggagagtgt

SEQ ID NO: 35 - protein, 107 aa, synthetic construct [sequence omitted]

SEQ ID NO: 36 - DNA, 321 bp, synthetic construct
  misc_feature 1..321: note = Description of Artificial Sequence: Synthetic polynucleotide
  source 1..321: mol_type = other DNA
gatattcagatgacccagtccccaagctccctgagtgcctcagtgggcgaccgagtcaccatcacatgcaaggcttcccaggatgtgtctattggagtcgcatggtaccagcagaagccaggcaaagcacccaagctgctgatctatagcgcctcctaccggtataccggcgtgccctctagattctctggcagtgggtcaggaacagactttactctgaccatctctagtctgcagcctgaggatttcgctacctactattgccagcagtactatatctacccatatacctttggccaggggacaaaagtggagatcaag

SEQ ID NO: 37 - protein, 6 aa, synthetic construct
  REGION 1..6: note = Description of Artificial Sequence: Synthetic peptide
QDVSIG

SEQ ID NO: 38 - DNA, 18 bp, synthetic construct
  misc_feature 1..18: note = Description of Artificial Sequence: Synthetic oligonucleotide
  source 1..18: mol_type = other DNA
caggatgtgtctattgga

SEQ ID NO: 39 - protein, 9 aa, synthetic construct
  REGION 1..9: note = Description of Artificial Sequence: Synthetic peptide
QQYYIYPYT

SEQ ID NO: 40 - DNA, 27 bp, synthetic construct
  misc_feature 1..27: note = Description of Artificial Sequence: Synthetic oligonucleotide
  source 1..27: mol_type = other DNA
cagcagtactatatctacccatatacc

SEQ ID NO: 41-42 - skipped (2 entries)

SEQ ID NO: 43 - protein, 107 aa, synthetic construct [sequence omitted]

SEQ ID NO: 44 - DNA, 321 bp, synthetic construct
  misc_feature 1..321: note = Description of Artificial Sequence: Synthetic polynucleotide
  source 1..321: mol_type = other DNA
aggactgtggccgctccctccgtcttcatttttcccccttctgacgaacagctgaaaagtggcacagccagcgtggtctgtctgctgaacaatttctaccctcgcgaagccaaagtgcagtggaaggtcgataacgctctgcagagcggcaacagccaggagtctgtgactgaacaggacagtaaagattcaacctatagcctgtcaagcacactgactctgagcaaggcagactacgagaagcacaaagtgtatgcctgcgaagtcacacatcaggggctgtcctctcctgtgactaagagctttaacagaggagagtgt

SEQ ID NO: 45 - protein, 222 aa, synthetic construct
  REGION 1..222: note = Description of Artificial Sequence: Synthetic polypeptide
DYKDDDDKDIQMTQSPSSLSASVGDRVTITCRASQDVNTAVAWYQQKPGKAPKLLIYSASFLYSGVPSRFSGSRSGTDFTLTISSLQPEDFATYYCQQHYTTPPTFGQGTKVEIKRTVAAPSVFIFPPSDERLKSGTASVVCLLNNFYPREAKVQWKVDNALQSGNSQESVTEQDSKDSTYSLSSTLTLSKADYEKHKVYACEVTHQGLSSPVTKSFNRGEC

SEQ ID NO: 46 - DNA, 666 bp, synthetic construct
  misc_feature 1..666: note = Description of Artificial Sequence: Synthetic polynucleotide
  source 1..666: mol_type = other DNA
gactacaaagacgacgatgacaaagatatccagatgacccagtcccctagctccctgtccgcttctgtgggcgatagggtcactattacctgccgcgcatctcaggacgtgaacaccgcagtcgcctggtaccagcagaagcctgggaaagctccaaagctgctgatctacagtgcatcattcctgtattcaggagtgcccagccggtttagcggcagcagatctggcaccgatttcacactgactatttctagtctgcagcctgaggactttgccacatactattgccagcagcactataccacaccccctactttcggccaggggaccaaagtggagatcaagcgaactgtggccgctccaagtgtcttcatttttccacccagcgatgaaagactgaagtccggcacagcttctgtggtctgtctgctgaacaatttttaccccagagaggccaaagtgcagtggaaggtcgacaacgctctgcagagtggcaacagccaggagagcgtgacagaacaggattccaaagactctacttatagtctgtcaagcaccctgacactgagcaaggcagactacgaaaagcataaagtgtatgcctgtgaggtcacacatcaggggctgtcatcaccagtcaccaaatcattcaatcggggggagtgc

SEQ ID NO: 47 - protein, 107 aa, synthetic construct [sequence omitted]

SEQ ID NO: 48 - DNA, 321 bp, synthetic construct
  misc_feature 1..321: note = Description of Artificial Sequence: Synthetic polynucleotide
  source 1..321: mol_type = other DNA
gatatccagatgacccagtcccctagctccctgtccgcttctgtgggcgatagggtcactattacctgccgcgcatctcaggacgtgaacaccgcagtcgcctggtaccagcagaagcctgggaaagctccaaagctgctgatctacagtgcatcattcctgtattcaggagtgcccagccggtttagcggcagcagatctggcaccgatttcacactgactatttctagtctgcagcctgaggactttgccacatactattgccagcagcactataccacaccccctactttcggccaggggaccaaagtggagatcaag

SEQ ID NO: 49 - protein, 6 aa, synthetic construct
  REGION 1..6: note = Description of Artificial Sequence: Synthetic peptide
QDVNTA

SEQ ID NO: 50 - DNA, 18 bp, synthetic construct
  misc_feature 1..18: note = Description of Artificial Sequence: Synthetic oligonucleotide
  source 1..18: mol_type = other DNA
caggacgtgaacaccgca

SEQ ID NO: 51 - protein, 9 aa, synthetic construct
  REGION 1..9: note = Description of Artificial Sequence: Synthetic peptide
QQHYTTPPT

SEQ ID NO: 52 - DNA, 27 bp, synthetic construct
  misc_feature 1..27: note = Description of Artificial Sequence: Synthetic oligonucleotide
  source 1..27: mol_type = other DNA
cagcagcactataccacaccccctact

SEQ ID NO: 53-54 - skipped (2 entries)

SEQ ID NO: 55 - protein, 107 aa, synthetic construct
  REGION 1..107: note = Description of Artificial Sequence: Synthetic polypeptide
RTVAAPSVFIFPPSDERLKSGTASVVCLLNNFYPREAKVQWKVDNALQSGNSQESVTEQDSKDSTYSLSSTLTLSKADYEKHKVYACEVTHQGLSSPVTKSFNRGEC

SEQ ID NO: 56 - DNA, 321 bp, synthetic construct
  misc_feature 1..321: note = Description of Artificial Sequence: Synthetic polynucleotide
  source 1..321: mol_type = other DNA
cgaactgtggccgctccaagtgtcttcatttttccacccagcgatgaaagactgaagtccggcacagcttctgtggtctgtctgctgaacaatttttaccccagagaggccaaagtgcagtggaaggtcgacaacgctctgcagagtggcaacagccaggagagcgtgacagaacaggattccaaagactctacttatagtctgtcaagcaccctgacactgagcaaggcagactacgaaaagcataaagtgtatgcctgtgaggtcacacatcaggggctgtcatcaccagtcaccaaatcattcaatcggggggagtgc

SEQ ID NO: 57 - protein, 222 aa, synthetic construct
  REGION 1..222: note = Description of Artificial Sequence: Synthetic polypeptide
DYKDDDDKDIQMTQSPSSLSASVGDRVTITCRASQDVNTAVAWYQQKPGKAPKLLIYSASFLYSGVPSRFSGSRSGTDFTLTISSLQPEDFATYYCQQHYTTPPTFGQGTKVEIKRTVAAPSVFIFPPSDERLKSGTASVVCLLNNFYPREAKVQWKVDNALQSGNSKESVTEQDSKDSTYSLSSRLTLSKADYEKHKVYACEVTHQGLSSPVTKSFNRGEC

SEQ ID NO: 58 - DNA, 666 bp, synthetic construct
  misc_feature 1..666: note = Description of Artificial Sequence: Synthetic polynucleotide
  source 1..666: mol_type = other DNA
gactacaaagacgacgatgacaaagatatccagatgacccagtcccctagctccctgtccgcttctgtgggcgatagggtcactattacctgccgcgcatctcaggacgtgaacaccgcagtcgcctggtaccagcagaagcctgggaaagctccaaagctgctgatctacagtgcatcattcctgtattcaggagtgcccagccggtttagcggcagcagatctggcaccgatttcacactgactatttctagtctgcagcctgaggactttgccacatactattgccagcagcactataccacaccccctactttcggccaggggaccaaagtggagatcaagcgaactgtggccgctccaagtgtcttcatttttccacccagcgatgaaagactgaagtccggcacagcttctgtggtctgtctgctgaacaatttttaccccagagaggccaaagtgcagtggaaggtcgacaacgctctgcagagtggcaacagcaaggagagcgtgacagaacaggattccaaagactctacttatagtctgtcaagcagactgacactgagcaaggcagactacgaaaagcataaagtgtatgcctgtgaggtcacacatcaggggctgtcatcaccagtcaccaaatcattcaatcggggggagtgc

SEQ ID NO: 59 - protein, 107 aa, synthetic construct [sequence omitted]

SEQ ID NO: 60 - DNA, 321 bp, synthetic construct; identical to SEQ ID NO: 48
  misc_feature 1..321: note = Description of Artificial Sequence: Synthetic polynucleotide
  source 1..321: mol_type = other DNA

SEQ ID NO: 61 - protein, 6 aa, synthetic construct
  REGION 1..6: note = Description of Artificial Sequence: Synthetic peptide
QDVNTA

SEQ ID NO: 62 - DNA, 18 bp, synthetic construct
  misc_feature 1..18: note = Description of Artificial Sequence: Synthetic oligonucleotide
  source 1..18: mol_type = other DNA
caggacgtgaacaccgca

SEQ ID NO: 63 - protein, 9 aa, synthetic construct
  REGION 1..9: note = Description of Artificial Sequence: Synthetic peptide
QQHYTTPPT

SEQ ID NO: 64 - DNA, 27 bp, synthetic construct
  misc_feature 1..27: note = Description of Artificial Sequence: Synthetic oligonucleotide
  source 1..27: mol_type = other DNA
cagcagcactataccacaccccctact

SEQ ID NO: 65-66 - skipped (2 entries)

SEQ ID NO: 67 - protein, 107 aa, synthetic construct
  REGION 1..107: note = Description of Artificial Sequence: Synthetic polypeptide
RTVAAPSVFIFPPSDERLKSGTASVVCLLNNFYPREAKVQWKVDNALQSGNSKESVTEQDSKDSTYSLSSRLTLSKADYEKHKVYACEVTHQGLSSPVTKSFNRGEC

SEQ ID NO: 68 - DNA, 321 bp, synthetic construct
  misc_feature 1..321: note = Description of Artificial Sequence: Synthetic polynucleotide
  source 1..321: mol_type = other DNA
cgaactgtggccgctccaagtgtcttcatttttccacccagcgatgaaagactgaagtccggcacagcttctgtggtctgtctgctgaacaatttttaccccagagaggccaaagtgcagtggaaggtcgacaacgctctgcagagtggcaacagcaaggagagcgtgacagaacaggattccaaagactctacttatagtctgtcaagcagactgacactgagcaaggcagactacgaaaagcataaagtgtatgcctgtgaggtcacacatcaggggctgtcatcaccagtcaccaaatcattcaatcggggggagtgc

SEQ ID NO: 69 - protein, 214 aa, synthetic construct
  REGION 1..214: note = Description of Artificial Sequence: Synthetic polypeptide
DIQMTQSPSSLSASVGDRVTITCKASQDVSIGVAWYQQKPGKAPKLLIYSASYRYTGVPSRFSGSGSGTDFTLTISSLQPEDFATYYCQQYYIYPATFGQGTKVEIKRTVAAPSVFIFPPSDEQLKSGTASVVCLLNNFYPREAKVQWKVDNALQSGNSQESVTEQDSKDSTYSLSSTLTLSKADYEKHKVYACEVTHQGLSSPVTKSFNRGEC

SEQ ID NO: 70 - DNA, 642 bp, synthetic construct
  misc_feature 1..642: note = Description of Artificial Sequence: Synthetic polynucleotide
  source 1..642: mol_type = other DNA
gatattcagatgacccagtccccaagctccctgagtgcctcagtgggcgaccgagtcaccatcacatgcaaggcttcccaggatgtgtctattggagtcgcatggtaccagcagaagccaggcaaagcacccaagctgctgatctatagcgcctcctaccggtataccggcgtgccctctagattctctggcagtgggtcaggaacagactttactctgaccatctctagtctgcagcctgaggatttcgctacctactattgccagcagtactatatctacccagccacctttggccaggggacaaaagtggagatcaagaggactgtggccgctccctccgtcttcatttttcccccttctgacgaacagctgaaaagtggcacagccagcgtggtctgtctgctgaacaatttctaccctcgcgaagccaaagtgcagtggaaggtcgataacgctctgcagagcggcaacagccaggagtctgtgactgaacaggacagtaaagattcaacctatagcctgtcaagcacactgactctgagcaaggcagactacgagaagcacaaagtgtatgcctgcgaagtcacacatcaggggctgtcctctcctgtgactaagagctttaacagaggagagtgt

SEQ ID NO: 71 - protein, 107 aa, synthetic construct
  REGION 1..107: note = Description of Artificial Sequence: Synthetic polypeptide
DIQMTQSPSSLSASVGDRVTITCKASQDVSIGVAWYQQKPGKAPKLLIYSASYRYTGVPSRFSGSGSGTDFTLTISSLQPEDFATYYCQQYYIYPATFGQGTKVEIK

SEQ ID NO: 72 - DNA, 321 bp, synthetic construct
  misc_feature 1..321: note = Description of Artificial Sequence: Synthetic polynucleotide
  source 1..321: mol_type = other DNA
gatattcagatgacccagtccccaagctccctgagtgcctcagtgggcgaccgagtcaccatcacatgcaaggcttcccaggatgtgtctattggagtcgcatggtaccagcagaagccaggcaaagcacccaagctgctgatctatagcgcctcctaccggtataccggcgtgccctctagattctctggcagtgggtcaggaacagactttactctgaccatctctagtctgcagcctgaggatttcgctacctactattgccagcagtactatatctacccagccacctttggccaggggacaaaagtggagatcaag

SEQ ID NO: 73 - protein, 6 aa, synthetic construct
  REGION 1..6: note = Description of Artificial Sequence: Synthetic peptide
QDVSIG

SEQ ID NO: 74 - DNA, 18 bp, synthetic construct
  misc_feature 1..18: note = Description of Artificial Sequence: Synthetic oligonucleotide
  source 1..18: mol_type = other DNA
caggatgtgtctattgga

SEQ ID NO: 75 - protein, 9 aa, synthetic construct
  REGION 1..9: note = Description of Artificial Sequence: Synthetic peptide
QQYYIYPAT

SEQ ID NO: 76 - DNA, 27 bp, synthetic construct
  misc_feature 1..27: note = Description of Artificial Sequence: Synthetic oligonucleotide
  source 1..27: mol_type = other DNA
cagcagtactatatctacccagccacc

SEQ ID NO: 77-78 - skipped (2 entries)

SEQ ID NO: 79 - protein, 107 aa, synthetic construct [sequence omitted]

SEQ ID NO: 80 - DNA, 321 bp, synthetic construct; identical to SEQ ID NO: 44
  misc_feature 1..321: note = Description of Artificial Sequence: Synthetic polynucleotide
  source 1..321: mol_type = other DNA

SEQ ID NO: 81 - protein, 449 aa, synthetic construct
  REGION 1..449: note = Description of Artificial Sequence: Synthetic polypeptide
EVQLVESGGGLVQPGGSLRLSCAASGFNIKDTYIHWVRQAPGKGLEWVARIYPTNGYTRYADSVKGRFTISADTSKNTAYLQMNSLRAEDTAVYYCSRWGGDGFYAMDYWGQGTLVTVSSASTKGPSVFPLAPSSKSTSGGTAALGCEVTDYFPEPVTVSWNSGALTSGVHTFPAVLQSSGLYSLSSVVTVPSSSLGTQTYICNVNHKPSNTKVDKKVEPKSCDKTHTCPPCPAPELLGGPSVFLFPPKPKDTLMISRTPEVTCVVVDVSHEDPEVKFNWYVDGVEVHNAKTKPREEQYNSTYRVVSVLTVLHQDWLNGKEYKCKVSNKALPAPIEKTISKAKGQPREPQVYVYPPSRDELTKNQVSLTCLVKGFYPSDIAVEWESNGQPENNYKTTPPVLDSDGSFALVSKLTVDKSRWQQGNVFSCSVMHEALHNHYTQKSLSLSPG

SEQ ID NO: 82 - DNA, 1347 bp, synthetic construct
  misc_feature 1..1347: note = Description of Artificial Sequence: Synthetic polynucleotide
  source 1..1347: mol_type = other DNA
gaggtgcagctggtcgaaagcggaggaggactggtgcagccaggagggtcactgcgactgagctgcgcagcttccggcttcaacatcaaggacacctacattcactgggtccgccaggctcctggaaaaggcctggagtgggtggcacgaatctatccaactaatggatacacccggtatgccgactccgtgaagggccggttcaccatttctgcagatacaagtaaaaacactgcctacctgcagatgaacagcctgcgagccgaagatacagccgtgtactattgcagccgatggggaggcgacggcttctacgctatggattattgggggcagggaaccctggtcacagtgagctccgcatcaacaaaggggcctagcgtgtttccactggccccctctagtaaatccacctctgggggaacagcagccctgggatgtgaggtgaccgactacttcccagagcccgtcactgtgagctggaactccggcgccctgacatctggggtccatacttttcctgctgtgctgcagtcaagcggcctgtacagcctgtcctctgtggtcactgtgccaagttcaagcctggggactcagacctatatctgcaacgtgaatcacaagccatccaataccaaagtcgacaagaaagtggaacccaagtcttgtgataaaacacatacttgccccccttgtcctgcaccagagctgctgggaggaccaagcgtgttcctgtttccacccaagcctaaagacaccctgatgattagtaggactccagaagtcacctgcgtggtcgtggacgtgagccacgaggaccccgaagtcaagttcaactggtacgtggatggcgtcgaggtgcataatgccaagacaaaacccagggaggaacagtacaactccacttatcgcgtcgtgtctgtcctgaccgtgctgcaccaggactggctgaacggcaaggagtataagtgcaaagtgagcaataaggctctgcccgcacctatcgagaaaacaatttccaaggctaaagggcagcctagagaaccacaggtgtacgtgtaccctccatctagggacgagctgaccaagaaccaggtcagtctgacatgtctggtgaaagggttctatcccagcgatatcgcagtggagtgggaatccaatggacagcctgagaacaattacaagaccacaccccctgtgctggactctgatggaagtttcgccctggtgagtaagctgaccgtcgataaatcacggtggcagcagggcaacgtgttcagctgttcagtgatgcacgaagcactgcacaaccactacacccagaaaagcctgtccctgtcccccggc

SEQ ID NO: 83 - protein, 120 aa, synthetic construct [sequence omitted]

SEQ ID NO: 84 - DNA, 360 bp, synthetic construct
  misc_feature 1..360: note = Description of Artificial Sequence: Synthetic polynucleotide
  source 1..360: mol_type = other DNA
gaggtgcagctggtcgaaagcggaggaggactggtgcagccaggagggtcactgcgactgagctgcgcagcttccggcttcaacatcaaggacacctacattcactgggtccgccaggctcctggaaaaggcctggagtgggtggcacgaatctatccaactaatggatacacccggtatgccgactccgtgaagggccggttcaccatttctgcagatacaagtaaaaacactgcctacctgcagatgaacagcctgcgagccgaagatacagccgtgtactattgcagccgatggggaggcgacggcttctacgctatggattattgggggcagggaaccctggtcacagtgagctcc

SEQ ID NO: 85 - protein, 8 aa, synthetic construct
  REGION 1..8: note = Description of Artificial Sequence: Synthetic peptide
GFNIKDTY

SEQ ID NO: 86 - DNA, 24 bp, synthetic construct
  misc_feature 1..24: note = Description of Artificial Sequence: Synthetic oligonucleotide
  source 1..24: mol_type = other DNA
ggcttcaacatcaaggacacctac

SEQ ID NO: 87 - protein, 13 aa, synthetic construct
  REGION 1..13: note = Description of Artificial Sequence: Synthetic peptide
SRWGGDGFYAMDY

SEQ ID NO: 88 - DNA, 39 bp, synthetic construct
  misc_feature 1..39: note = Description of Artificial Sequence: Synthetic oligonucleotide
  source 1..39: mol_type = other DNA
agccgatggggaggcgacggcttctacgctatggattat

SEQ ID NO: 89 - protein, 8 aa, synthetic construct
  REGION 1..8: note = Description of Artificial Sequence: Synthetic peptide
IYPTNGYT

SEQ ID NO: 90 - DNA, 24 bp, synthetic construct
  misc_feature 1..24: note = Description of Artificial Sequence: Synthetic oligonucleotide
  source 1..24: mol_type = other DNA
atctatccaactaatggatacacc

SEQ ID NO: 91 - protein, 98 aa, synthetic construct
  REGION 1..98: note = Description of Artificial Sequence: Synthetic polypeptide
ASTKGPSVFPLAPSSKSTSGGTAALGCEVTDYFPEPVTVSWNSGALTSGVHTFPAVLQSSGLYSLSSVVTVPSSSLGTQTYICNVNHKPSNTKVDKKV

SEQ ID NO: 92 - DNA, 294 bp, synthetic construct
  misc_feature 1..294: note = Description of Artificial Sequence: Synthetic polynucleotide
  source 1..294: mol_type = other DNA
gcatcaacaaaggggcctagcgtgtttccactggccccctctagtaaatccacctctgggggaacagcagccctgggatgtgaggtgaccgactacttcccagagcccgtcactgtgagctggaactccggcgccctgacatctggggtccatacttttcctgctgtgctgcagtcaagcggcctgtacagcctgtcctctgtggtcactgtgccaagttcaagcctggggactcagacctatatctgcaacgtgaatcacaagccatccaataccaaagtcgacaagaaagtg

SEQ ID NO: 93 - protein, 110 aa, synthetic construct; identical to SEQ ID NO: 13
  REGION 1..110: note = Description of Artificial Sequence: Synthetic polypeptide

SEQ ID NO: 94 - DNA, 330 bp, synthetic construct
  misc_feature 1..330: note = Description of Artificial Sequence: Synthetic polynucleotide
  source 1..330: mol_type = other DNA
gcaccagagctgctgggaggaccaagcgtgttcctgtttccacccaagcctaaagacaccctgatgattagtaggactccagaagtcacctgcgtggtcgtggacgtgagccacgaggaccccgaagtcaagttcaactggtacgtggatggcgtcgaggtgcataatgccaagacaaaacccagggaggaacagtacaactccacttatcgcgtcgtgtctgtcctgaccgtgctgcaccaggactggctgaacggcaaggagtataagtgcaaagtgagcaataaggctctgcccgcacctatcgagaaaacaatttccaaggctaaa

SEQ ID NO: 95 - protein, 106 aa, synthetic construct
  REGION 1..106: note = Description of Artificial Sequence: Synthetic polypeptide
GQPREPQVYVYPPSRDELTKNQVSLTCLVKGFYPSDIAVEWESNGQPENNYKTTPPVLDSDGSFALVSKLTVDKSRWQQGNVFSCSVMHEALHNHYTQKSLSLSPG

SEQ ID NO: 96 - DNA, 318 bp, synthetic construct
  misc_feature 1..318: note = Description of Artificial Sequence: Synthetic polynucleotide
  source 1..318: mol_type = other DNA
gggcagcctagagaaccacaggtgtacgtgtaccctccatctagggacgagctgaccaagaaccaggtcagtctgacatgtctggtgaaagggttctatcccagcgatatcgcagtggagtgggaatccaatggacagcctgagaacaattacaagaccacaccccctgtgctggactctgatggaagtttcgccctggtgagtaagctgaccgtcgataaatcacggtggcagcagggcaacgtgttcagctgttcagtgatgcacgaagcactgcacaaccactacacccagaaaagcctgtccctgtcccccggc

SEQ ID NO: 97 - protein, 448 aa, synthetic construct
  REGION 1..448: note = Description of Artificial Sequence: Synthetic polypeptide
EVQLVESGGGLVQPGGSLRLSCAASGFTFADYTMDWVRQAPGKGLEWVGDVNPNSGGSIYNQRFKGRFTFSVDRSKNTLYLQMNSLRAEDTAVYYCARNLGPSFYFDYWGQGTLVTVSSASTKGPSVFPLAPSSKSTSGGTAALGCLVKDYFPEPVTVSWNSGALTSGVHTFPAVLQSSGLYSLSSVVTVPSSSLGTQTYICNVNHKPSNTKVDKKVEPKSCDKTHTCPPCPAPELLGGPSVFLFPPKPKDTLMISRTPEVTCVVVDVSHEDPEVKFNWYVDGVEVHNAKTKPREEQYNSTYRVVSVLTVLHQDWLNGKEYKCKVSNKALPAPIEKTISKAKGQPREPQVYVYPPSRDELTKNQVSLTCLVKGFYPSDIAVEWESNGQPENNYKTTPPVLDSDGSFALVSKLTVDKSRWQQGNVFSCSVMHEALHNHYTQKSLSLSPG

SEQ ID NO: 98 - DNA, 1344 bp, synthetic construct
  misc_feature 1..1344: note = Description of Artificial Sequence: Synthetic polynucleotide
  source 1..1344: mol_type = other DNA
gaggtgcagctggtggaatcaggagggggcctggtgcagcccggagggtctctgcgactgtcatgtgccgcttctgggttcactttcgcagactacacaatggattgggtgcgacaggcccccggaaagggactggagtgggtgggcgatgtcaaccctaattctggcgggagtatctacaaccagcggttcaaggggagattcactttttcagtggacagaagcaaaaacaccctgtatctgcagatgaacagcctgagggccgaagataccgctgtctactattgcgctcgcaatctgggccccagtttctactttgactattgggggcagggaaccctggtgacagtcagctccgctagcactaaggggccttccgtgtttccactggctccctctagtaaatccacctctggaggcacagctgcactgggatgtctggtgaaggattacttccctgaaccagtcacagtgagttggaactcaggggctctgacaagtggagtccatacttttcccgcagtgctgcagtcaagcggactgtactccctgtcctctgtggtcaccgtgcctagttcaagcctgggcacccagacatatatctgcaacgtgaatcacaagccatcaaatacaaaagtcgacaagaaagtggagcccaagagctgtgataaaactcatacctgcccaccttgtccggcgccagaactgctgggaggaccaagcgtgttcctgtttccacccaagcctaaagacaccctgatgatttcccggactcctgaggtcacctgcgtggtcgtggacgtgtctcacgaggaccccgaagtcaagttcaactggtacgtggatggcgtcgaagtgcataatgccaagaccaaaccccgggaggaacagtacaactctacctatagagtcgtgagtgtcctgacagtgctgcaccaggactggctgaatgggaaggagtataagtgtaaagtgagcaacaaagccctgcccgccccaatcgaaaaaacaatctctaaagcaaaaggacagcctcgcgaaccacaggtctacgtctaccccccatcaagagatgaactgacaaaaaatcaggtctctctgacatgcctggtcaaaggattctacccttccgacatcgccgtggagtgggaaagtaacggccagcccgagaacaattacaagaccacaccccctgtcctggactctgatgggagtttcgctctggtgtcaaagctgaccgtcgataaaagccggtggcagcagggcaatgtgtttagctgctccgtcatgcacgaagccctgcacaatcactacacacagaagtccctgagcctgagccctggc

SEQ ID NO: 99 - protein, 119 aa, synthetic construct
  REGION 1..119: note = Description of Artificial Sequence: Synthetic polypeptide
EVQLVESGGGLVQPGGSLRLSCAASGFTFADYTMDWVRQAPGKGLEWVGDVNPNSGGSIYNQRFKGRFTFSVDRSKNTLYLQMNSLRAEDTAVYYCARNLGPSFYFDYWGQGTLVTVSS

SEQ ID NO: 100 - DNA, 357 bp, synthetic construct
  misc_feature 1..357: note = Description of Artificial Sequence: Synthetic polynucleotide
  source 1..357: mol_type = other DNA
gaggtgcagctggtggaatcaggagggggcctggtgcagcccggagggtctctgcgactgtcatgtgccgcttctgggttcactttcgcagactacacaatggattgggtgcgacaggcccccggaaagggactggagtgggtgggcgatgtcaaccctaattctggcgggagtatctacaaccagcggttcaaggggagattcactttttcagtggacagaagcaaaaacaccctgtatctgcagatgaacagcctgagggccgaagataccgctgtctactattgcgctcgcaatctgggccccagtttctactttgactattgggggcagggaaccctggtgacagtcagctcc

SEQ ID NO: 101 - protein, 8 aa, synthetic construct
  REGION 1..8: note = Description of Artificial Sequence: Synthetic peptide
GFTFADYT

SEQ ID NO: 102 - DNA, 24 bp, synthetic construct
  misc_feature 1..24: note = Description of Artificial Sequence: Synthetic oligonucleotide
  source 1..24: mol_type = other DNA
gggttcactttcgcagactacaca

SEQ ID NO: 103 - protein, 12 aa, synthetic construct
  REGION 1..12: note = Description of Artificial Sequence: Synthetic peptide
ARNLGPSFYFDY

SEQ ID NO: 104 - DNA, 36 bp, synthetic construct
  misc_feature 1..36: note = Description of Artificial Sequence: Synthetic oligonucleotide
  source 1..36: mol_type = other DNA
gctcgcaatctgggccccagtttctactttgactat

SEQ ID NO: 105 - protein, 8 aa, synthetic construct
  REGION 1..8: note = Description of Artificial Sequence: Synthetic peptide
VNPNSGGS

SEQ ID NO: 106 - DNA, 24 bp, synthetic construct
  misc_feature 1..24: note = Description of Artificial Sequence: Synthetic oligonucleotide
  source 1..24: mol_type = other DNA
gtcaaccctaattctggcgggagt

SEQ ID NO: 107 - protein, 98 aa, synthetic construct; identical to SEQ ID NO: 11
  REGION 1..98: note = Description of Artificial Sequence: Synthetic polypeptide

SEQ ID NO: 108 - DNA, 294 bp, synthetic construct
  misc_feature 1..294: note = Description of Artificial Sequence: Synthetic polynucleotide
  source 1..294: mol_type = other DNA
gctagcactaaggggccttccgtgtttccactggctccctctagtaaatccacctctggaggcacagctgcactgggatgtctggtgaaggattacttccctgaaccagtcacagtgagttggaactcaggggctctgacaagtggagtccatacttttcccgcagtgctgcagtcaagcggactgtactccctgtcctctgtggtcaccgtgcctagttcaagcctgggcacccagacatatatctgcaacgtgaatcacaagccatcaaatacaaaagtcgacaagaaagtg

SEQ ID NO: 109 - protein, 110 aa, synthetic construct; identical to SEQ ID NO: 13
  REGION 1..110: note = Description of Artificial Sequence: Synthetic polypeptide

SEQ ID NO: 110 - DNA, 330 bp, synthetic construct
  misc_feature 1..330: note = Description of Artificial Sequence: Synthetic polynucleotide
  source 1..330: mol_type = other DNA
gcgccagaactgctgggaggaccaagcgtgttcctgtttccacccaagcctaaagacaccctgatgatttcccggactcctgaggtcacctgcgtggtcgtggacgtgtctcacgaggaccccgaagtcaagttcaactggtacgtggatggcgtcgaagtgcataatgccaagaccaaaccccgggaggaacagtacaactctacctatagagtcgtgagtgtcctgacagtgctgcaccaggactggctgaatgggaaggagtataagtgtaaagtgagcaacaaagccctgcccgccccaatcgaaaaaacaatctctaaagcaaaa

SEQ ID NO: 111 - protein, 106 aa, synthetic construct; identical to SEQ ID NO: 95
  REGION 1..106: note = Description of Artificial Sequence: Synthetic polypeptide

SEQ ID NO: 112 - DNA, 318 bp, synthetic construct
  misc_feature 1..318: note = Description of Artificial Sequence: Synthetic polynucleotide
  source 1..318: mol_type = other DNA
ggacagcctcgcgaaccacaggtctacgtctaccccccatcaagagatgaactgacaaaaaatcaggtctctctgacatgcctggtcaaaggattctacccttccgacatcgccgtggagtgggaaagtaacggccagcccgagaacaattacaagaccacaccccctgtcctggactctgatgggagtttcgctctggtgtcaaagctgaccgtcgataaaagccggtggcagcagggcaatgtgtttagctgctccgtcatgcacgaagccctgcacaatcactacacacagaagtccctgagcctgagccctggc

SEQ ID NO: 113 - protein, 226 aa, synthetic construct
  REGION 1..226: note = Description of Artificial Sequence: Synthetic polypeptide
YPYDVPDYATGSDIQMTQSPSSLSASVGDRVTITCKASQDVSIGVAWYQQKPGKAPKLLIYSASYRYTGVPSRFSGSGSGTDFTLTISSLQPEDFATYYCQQYYIYPYTFGQGTKVEIKRTVAAPSVFIFPPSDEELKSGTASVVCLLNNFYPREAKVQWKVDNALQSGNSEESVTEQDSKDSTYSLSSTLELSKADYEKHKVYACEVTHQGLSSPVTKSFNRGEC

SEQ ID NO: 114 - DNA, 678 bp, synthetic construct
  misc_feature 1..678: note = Description of Artificial Sequence: Synthetic polynucleotide
  source 1..678: mol_type = other DNA
tatccctacgatgtgcctgactacgctactggctccgatatccagatgacccagtctccaagctccctgagtgcatcagtgggggaccgagtcaccatcacatgcaaggcttcccaggatgtgtctattggagtcgcatggtaccagcagaagccaggcaaagcacccaagctgctgatctacagcgcctcctaccggtatactggggtgccttccagattctctggcagtgggtcaggaaccgactttactctgaccatctctagtctgcagcccgaggatttcgccacctactattgccagcagtactatatctacccttatacctttggccaggggacaaaagtggagatcaagaggacagtggccgctccaagtgtcttcatttttcccccttccgacgaagagctgaaaagtggaactgcttcagtggtctgtctgctgaacaatttctacccccgcgaagccaaagtgcagtggaaggtcgataacgctctgcagagcggcaattccgaggagtctgtgacagaacaggacagtaaagattcaacttatagcctgtcaagcacactggagctgtctaaggcagactacgagaagcacaaagtgtatgcctgcgaagtcacccatcaggggctgtcctctcccgtgacaaagagctttaacagaggagagtgt

SEQ ID NO: 115 - protein, 107 aa, synthetic construct [sequence omitted]

SEQ ID NO: 116 - DNA, 321 bp, synthetic construct
  misc_feature 1..321: note = Description of Artificial Sequence: Synthetic polynucleotide
  source 1..321: mol_type = other DNA
gatatccagatgacccagtctccaagctccctgagtgcatcagtgggggaccgagtcaccatcacatgcaaggcttcccaggatgtgtctattggagtcgcatggtaccagcagaagccaggcaaagcacccaagctgctgatctacagcgcctcctaccggtatactggggtgccttccagattctctggcagtgggtcaggaaccgactttactctgaccatctctagtctgcagcccgaggatttcgccacctactattgccagcagtactatatctacccttatacctttggccaggggacaaaagtggagatcaag

SEQ ID NO: 117 - protein, 6 aa, synthetic construct
  REGION 1..6: note = Description of Artificial Sequence: Synthetic peptide
QDVSIG

SEQ ID NO: 118 - DNA, 18 bp, synthetic construct
  misc_feature 1..18: note = Description of Artificial Sequence: Synthetic oligonucleotide
  source 1..18: mol_type = other DNA
caggatgtgtctattgga

SEQ ID NO: 119 - protein, 9 aa, synthetic construct
  REGION 1..9: note = Description of Artificial Sequence: Synthetic peptide
QQYYIYPYT

SEQ ID NO: 120 - DNA, 27 bp, synthetic construct
  misc_feature 1..27: note = Description of Artificial Sequence: Synthetic oligonucleotide
  source 1..27: mol_type = other DNA
cagcagtactatatctacccttatacc

SEQ ID NO: 121-122 - skipped (2 entries)

SEQ ID NO: 123 - protein, 107 aa, synthetic construct
  REGION 1..107: note = Description of Artificial Sequence: Synthetic polypeptide
RTVAAPSVFIFPPSDEELKSGTASVVCLLNNFYPREAKVQWKVDNALQSGNSEESVTEQDSKDSTYSLSSTLELSKADYEKHKVYACEVTHQGLSSPVTKSFNRGEC

SEQ ID NO: 124 - DNA, 321 bp, synthetic construct
  misc_feature 1..321: note = Description of Artificial Sequence: Synthetic polynucleotide
  source 1..321: mol_type = other DNA
aggacagtggccgctccaagtgtcttcatttttcccccttccgacgaagagctgaaaagtggaactgcttcagtggtctgtctgctgaacaatttctacccccgcgaagccaaagtgcagtggaaggtcgataacgctctgcagagcggcaattccgaggagtctgtgacagaacaggacagtaaagattcaacttatagcctgtcaagcacactggagctgtctaaggcagactacgagaagcacaaagtgtatgcctgcgaagtcacccatcaggggctgtcctctcccgtgacaaagagctttaacagaggagagtgt

SEQ ID NO: 125 - protein, 450 aa, synthetic construct
  REGION 1..450: note = Description of Artificial Sequence: Synthetic polypeptide
EVQLVESGGGLVQPGGSLRLSCAASGFNIKDTYIHWVRQAPGKGLEWVARIYPTNGYTRYADSVKGRFTISADTSKNTAYLQMNSLRAEDTAVYYCSRWGGDGFYAMDYWGQGTLVTVSSASTKGPSVFPLAPSSKSTSGGTAALGCLVKDYFPEPVTVSWNSGALTSGVHTFPAVLQSSGLYSLSSVVTVPSSSLGTQTYICNVNHKPSNTKVDKKVEPKSCDKTHTCPPCPAPELLGGPSVFLFPPKPKDTLMISRTPEVTCVVVDVSHEDPEVKFNWYVDGVEVHNAKTKPREEQYNSTYRVVSVLTVLHQDWLNGKEYKCKVSNKALPAPIEKTISKAKGQPREPQVYVYPPSRDELTKNQVSLTCLVKGFYPSDIAVEWESNGQPENNYKTTPPVLDSDGSFALVSKLTVDKSRWQQGNVFSCSVMHEALHNHYTQKSLSLSPGK

SEQ ID NO: 126 - DNA, 1350 bp, synthetic construct
  misc_feature 1..1350: note = Description of Artificial Sequence: Synthetic polynucleotide
  source 1..1350: mol_type = other DNA
gaagtccagctggtcgaaagcggaggaggactggtgcagccaggagggtctctgcgactgagttgcgccgcttcaggcttcaacatcaaggacacctacattcactgggtgcgccaggctcctggaaaaggcctggagtgggtggcacgaatctatccaactaatggatacacccggtatgcagacagcgtgaagggccggttcaccattagcgcagatacatccaaaaacactgcctacctgcagatgaacagcctgcgagccgaagatactgctgtgtactattgcagtcggtggggaggcgacggcttctacgctatggattattgggggcagggaaccctggtcacagtgagctccgcatctacaaaggggcctagtgtgtttccactggccccctctagtaaatccacctctgggggaacagcagccctgggatgtctggtgaaggactatttcccagagcccgtcactgtgagttggaactcaggcgccctgacatccggggtccatacttttcctgctgtgctgcagtcaagcggcctgtactctctgtcctctgtggtcaccgtgccaagttcaagcctggggactcagacctatatctgcaacgtgaatcacaagccaagcaatacaaaagtcgacaagaaagtggaacccaagagctgtgataaaacacatacttgccccccttgtcctgcaccagagctgctgggaggaccatccgtgttcctgtttccacccaagcctaaagacaccctgatgatttccaggactccagaagtcacctgcgtggtcgtggacgtgtctcacgaggaccccgaagtcaagttcaactggtacgtggatggcgtcgaggtgcataatgccaagacaaaacccagggaggaacagtacaactcaacttatcgcgtcgtgagcgtcctgaccgtgctgcaccaggactggctgaacggcaaggagtataagtgcaaagtgagcaataaggctctgcccgcacctatcgagaaaaccattagcaaggccaaagggcagcctagagaaccacaggtctacgtgtatcctccaagcagggacgagctgaccaagaaccaggtctccctgacatgtctggtgaaagggttttaccccagtgatatcgctgtggagtgggaatcaaatggacagcctgaaaacaattataagaccacaccccctgtgctggacagcgatggcagcttcgctctggtctccaagctgactgtggataaatctcggtggcagcagggcaacgtctttagttgttcagtgatgcatgaggcactgcacaatcattacacccagaagagcctgtccctgtctcccggcaaa

SEQ ID NO: 127 - protein, 120 aa, synthetic construct [sequence omitted]

SEQ ID NO: 128 - DNA, 360 bp, synthetic construct
  misc_feature 1..360: note = Description of Artificial Sequence: Synthetic polynucleotide
  source 1..360: mol_type = other DNA
gaagtccagctggtcgaaagcggaggaggactggtgcagccaggagggtctctgcgactgagttgcgccgcttcaggcttcaacatcaaggacacctacattcactgggtgcgccaggctcctggaaaaggcctggagtgggtggcacgaatctatccaactaatggatacacccggtatgcagacagcgtgaagggccggttcaccattagcgcagatacatccaaaaacactgcctacctgcagatgaacagcctgcgagccgaagatactgctgtgtactattgcagtcggtggggaggcgacggcttctacgctatggattattgggggcagggaaccctggtcacagtgagctcc

SEQ ID NO: 129 - protein, 8 aa, synthetic construct
  REGION 1..8: note = Description of Artificial Sequence: Synthetic peptide
GFNIKDTY

SEQ ID NO: 130 - DNA, 24 bp, synthetic construct
  misc_feature 1..24: note = Description of Artificial Sequence: Synthetic oligonucleotide
  source 1..24: mol_type = other DNA
ggcttcaacatcaaggacacctac

SEQ ID NO: 131 - protein, 13 aa, synthetic construct
  REGION 1..13: note = Description of Artificial Sequence: Synthetic peptide
SRWGGDGFYAMDY

SEQ ID NO: 132 - DNA, 39 bp, synthetic construct
  misc_feature 1..39: note = Description of Artificial Sequence: Synthetic oligonucleotide
  source 1..39: mol_type = other DNA
agtcggtggggaggcgacggcttctacgctatggattat

SEQ ID NO: 133 - protein, 8 aa, synthetic construct
  REGION 1..8: note = Description of Artificial Sequence: Synthetic peptide
IYPTNGYT

SEQ ID NO: 134 - DNA, 24 bp, synthetic construct
  misc_feature 1..24: note = Description of Artificial Sequence: Synthetic oligonucleotide
  source 1..24: mol_type = other DNA
atctatccaactaatggatacacc

SEQ ID NO: 135 - protein, 98 aa, synthetic construct; identical to SEQ ID NO: 11
  REGION 1..98: note = Description of Artificial Sequence: Synthetic polypeptide

SEQ ID NO: 136 - DNA, 294 bp, synthetic construct
  misc_feature 1..294: note = Description of Artificial Sequence: Synthetic polynucleotide
  source 1..294: mol_type = other DNA
gcatctacaaaggggcctagtgtgtttccactggccccctctagtaaatccacctctgggggaacagcagccctgggatgtctggtgaaggactatttcccagagcccgtcactgtgagttggaactcaggcgccctgacatccggggtccatacttttcctgctgtgctgcagtcaagcggcctgtactctctgtcctctgtggtcaccgtgccaagttcaagcctggggactcagacctatatctgcaacgtgaatcacaagccaagcaatacaaaagtcgacaagaaagtg

SEQ ID NO: 137 - protein, 110 aa, synthetic construct; identical to SEQ ID NO: 13
  REGION 1..110: note = Description of Artificial Sequence: Synthetic polypeptide

SEQ ID NO: 138 - DNA, 330 bp, synthetic construct
  misc_feature 1..330: note = Description of Artificial Sequence: Synthetic polynucleotide
  source 1..330: mol_type = other DNA
gcaccagagctgctgggaggaccatccgtgttcctgtttccacccaagcctaaagacaccctgatgatttccaggactccagaagtcacctgcgtggtcgtggacgtgtctcacgaggaccccgaagtcaagttcaactggtacgtggatggcgtcgaggtgcataatgccaagacaaaacccagggaggaacagtacaactcaacttatcgcgtcgtgagcgtcctgaccgtgctgcaccaggactggctgaacggcaaggagtataagtgcaaagtgagcaataaggctctgcccgcacctatcgagaaaaccattagcaaggccaaa

SEQ ID NO: 139 - protein, 106 aa, synthetic construct; identical to SEQ ID NO: 95
  REGION 1..106: note = Description of Artificial Sequence: Synthetic polypeptide

SEQ ID NO: 140 - DNA, 318 bp, synthetic construct
  misc_feature 1..318: note = Description of Artificial Sequence: Synthetic polynucleotide
  source 1..318: mol_type = other DNA
gggcagcctagagaaccacaggtctacgtgtatcctccaagcagggacgagctgaccaagaaccaggtctccctgacatgtctggtgaaagggttttaccccagtgatatcgctgtggagtgggaatcaaatggacagcctgaaaacaattataagaccacaccccctgtgctggacagcgatggcagcttcgctctggtctccaagctgactgtggataaatctcggtggcagcagggcaacgtctttagttgttcagtgatgcatgaggcactgcacaatcattacacccagaagagcctgtccctgtctcccggc

SEQ ID NO: 141 - protein, 232 aa, synthetic construct
  REGION 1..232: note = Description of Artificial Sequence: Synthetic polypeptide
EPKSSDKTHTCPPCPAPELLGGPSVFLFPPKPKDTLMISRTPEVTCVVVDVSHEDPEVKFNWYVDGVEVHNAKTKPREEQYNSTYRVVSVLTVLHQDWLNGKEYKCKVSNKALPAPIEKTISKAKGQPREPQVYTLPPSRDELTKNQVSLICLVKGFYPSDIAVEWESNGQPENRYMTWPPVLDSDGSFFLYSKLTVDKSRWQQGNVFSCSVMHEALHNHYTQKSLSLSPGK

SEQ ID NO: 142 - DNA, 696 bp, synthetic construct
  misc_feature 1..696: note = Description of Artificial Sequence: Synthetic polynucleotide
  source 1..696: mol_type = other DNA
gagcccaagagcagcgataagacccacacctgccctccctgtccagctccagaactgctgggaggacctagcgtgttcctgtttccccctaagccaaaagacactctgatgatttccaggactcccgaggtgacctgcgtggtggtggacgtgtctcacgaggaccccgaagtgaagttcaactggtacgtggatggcgtggaagtgcataatgctaagacaaaaccaagagaggaacagtacaactccacttatcgcgtcgtgagcgtgctgaccgtgctgcaccaggactggctgaacgggaaggagtataagtgcaaagtcagtaataaggccctgcctgctccaatcgaaaaaaccatctctaaggccaaaggccagccaagggagccccaggtgtacacactgccacccagcagagacgaactgaccaagaaccaggtgtccctgatctgtctggtgaaaggcttctatcctagtgatattgctgtggagtgggaatcaaatggacagccagagaacagatacatgacctggcctccagtgctggacagcgatggcagcttcttcctgtattccaagctgacagtggataaatctcgatggcagcaggggaacgtgtttagttgttcagtgatgcatgaagccctgcacaatcattacactcagaagagcctgtccctgtctcccggcaaa

SEQ ID NO: 143 - protein, 110 aa, synthetic construct; identical to SEQ ID NO: 13
  REGION 1..110: note = Description of Artificial Sequence: Synthetic polypeptide

SEQ ID NO: 144 - DNA, 330 bp, synthetic construct; identical to SEQ ID NO: 14
  misc_feature 1..330: note = Description of Artificial Sequence: Synthetic polynucleotide
  source 1..330: mol_type = other DNA

SEQ ID NO: 145 - protein, 106 aa, synthetic construct
  REGION 1..106: note = Description of Artificial Sequence: Synthetic polypeptide
GQPREPQVYTLPPSRDELTKNQVSLICLVKGFYPSDIAVEWESNGQPENRYMTWPPVLDSDGSFFLYSKLTVDKSRWQQGNVFSCSVMHEALHNHYTQKSLSLSPG

SEQ ID NO: 146 - DNA, 318 bp, synthetic construct
  misc_feature 1..318: note = Description of Artificial Sequence: Synthetic polynucleotide
  source 1..318: mol_type = other DNA
ggccagccaagggagccccaggtgtacacactgccacccagcagagacgaactgaccaagaaccaggtgtccctgatctgtctggtgaaaggcttctatcctagtgatattgctgtggagtgggaatcaaatggacagccagagaacagatacatgacctggcctccagtgctggacagcgatggcagcttcttcctgtattccaagctgacagtggataaatctcgatggcagcaggggaacgtgtttagttgttcagtgatgcatgaagccctgcacaatcattacactcagaagagcctgtccctgtctcccggc

SEQ ID NO: 147 - protein, 481 aa, synthetic construct
  REGION 1..481: note = Description of Artificial Sequence: Synthetic polypeptide
DIQMTQSPSSLSASVGDRVTITCRASQDVNTAVAWYQQKPGKAPKLLIYSASFLYSGVPSRFSGSRSGTDFTLTISSLQPEDFATYYCQQHYTTPPTFGQGTKVEIKGGSGGGSGGGSGGGSGGGSGEVQLVESGGGLVQPGGSLRLSCAASGFNIKDTYIHWVRQAPGKGLEWVARIYPTNGYTRYADSVKGRFTISADTSKNTAYLQMNSLRAEDTAVYYCSRWGGDGFYAMDYWGQGTLVTVSSAAEPKSSDKTHTCPPCPAPELLGGPSVFLFPPKPKDTLMISRTPEVTCVVVDVSHEDPEVKFNWYVDGVEVHNAKTKPREEQYNSTYRVVSVLTVLHQDWLNGKEYKCKVSNKALPAPIEKTISKAKGQPREPQVYTYPPSRDELTKNQVSLTCLVKGFYPSDIAVEWESNGQPENNYKTTPPVLDEDGSFALVSKLTVDKSRWQQGNVFSCSVMHEALHNHYTQKSLSLSPGK

SEQ ID NO: 148 - DNA, 1443 bp, synthetic construct
  misc_feature 1..1443: note = Description of Artificial Sequence: Synthetic polynucleotide
  source 1..1443: mol_type = other DNA
gacatccagatgacccagtctccatcctccctgtctgcatctgtaggagacagagtcaccatcacttgccgggcaagtcaggacgttaacaccgctgtagcttggtatcagcagaaaccagggaaagcccctaagctcctgatctattctgcatcctttttgtacagtggggtcccatcaaggttcagtggcagtcgatctgggacagatttcactctcaccatcagcagtctgcaacctgaagattttgcaacttactactgtcaacagcattacactaccccacccactttcggccaagggaccaaagtggagatcaaaggtggttctggtggtggttctggtggtggttctggtggtggttctggtggtggttctggtgaagtgcagctggtggagtctgggggaggcttggtacagcctggcgggtccctgagactctcctgtgcagcctctggattcaacattaaagatacttatatccactgggtccggcaagctccagggaagggcctggagtgggtcgcacgtatttatcccacaaatggttacacacggtatgcggactctgtgaagggccgattcaccatctccgcagacacttccaagaacaccgcgtatctgcaaatgaacagtctgagagctgaggacacggccgtttattactgttcaagatggggcggagacggtttctacgctatggactactggggccaagggaccctggtcaccgtctcctcagccgccgagcccaagagcagcgataagacccacacctgccctccctgtccagctccagaactgctgggaggacctagcgtgttcctgtttccccctaagccaaaagacactctgatgatttccaggactcccgaggtgacctgcgtggtggtggacgtgtctcacgaggaccccgaagtgaagttcaactggtacgtggatggcgtggaagtgcataatgctaagacaaaaccaagagaggaacagtacaactccacttatcgcgtcgtgagcgtgctgaccgtgctgcaccaggactggctgaacgggaaggagtataagtgcaaagtcagtaataaggccctgcctgctccaatcgaaaaaaccatctctaaggccaaaggccagccaagggagccccaggtgtacacatacccacccagcagagacgaactgaccaagaaccaggtgtccctgacatgtctggtgaaaggcttctatcctagtgatattgctgtggagtgggaatcaaatggacagccagagaacaattacaagaccacacctccagtgctggacgaggatggcagcttcgccctggtgtccaagctgacagtggataaatctcgatggcagcaggggaacgtgtttagttgttcagtgatgcatgaagccctgcacaatcattacactcagaagagcctgtccctgtctcccggcaaa

SEQ ID NO: 149 - protein, 107 aa, synthetic construct [sequence omitted]

SEQ ID NO: 150 - DNA, 321 bp, synthetic construct
  misc_feature 1..321: note = Description of Artificial Sequence: Synthetic polynucleotide
  source 1..321: mol_type = other DNA
gacatccagatgacccagtctccatcctccctgtctgcatctgtaggagacagagtcaccatcacttgccgggcaagtcaggacgttaacaccgctgtagcttggtatcagcagaaaccagggaaagcccctaagctcctgatctattctgcatcctttttgtacagtggggtcccatcaaggttcagtggcagtcgatctgggacagatttcactctcaccatcagcagtctgcaacctgaagattttgcaacttactactgtcaacagcattacactaccccacccactttcggccaagggaccaaagtggagatcaaa

SEQ ID NO: 151 - protein, 6 aa, synthetic construct
  REGION 1..6: note = Description of Artificial Sequence: Synthetic peptide
QDVNTA

SEQ ID NO: 152 - DNA, 18 bp, synthetic construct
  misc_feature 1..18: note = Description of Artificial Sequence: Synthetic oligonucleotide
  source 1..18: mol_type = other DNA
caggacgttaacaccgct

SEQ ID NO: 153 - protein, 9 aa, synthetic construct
  REGION 1..9: note = Description of Artificial Sequence: Synthetic peptide
QQHYTTPPT

SEQ ID NO: 154 - DNA, 27 bp, synthetic construct
  misc_feature 1..27: note = Description of Artificial Sequence: Synthetic oligonucleotide
  source 1..27: mol_type = other DNA
caacagcattacactaccccacccact

SEQ ID NO: 155-156 - skipped (2 entries)

SEQ ID NO: 157 - protein, 120 aa, synthetic construct [sequence omitted]

SEQ ID NO: 158 - DNA, 360 bp, synthetic construct
  misc_feature 1..360: note = Description of Artificial Sequence: Synthetic polynucleotide
  source 1..360: mol_type = other DNA
gaagtgcagctggtggagtctgggggaggcttggtacagcctggcgggtccctgagactctcctgtgcagcctctggattcaacattaaagatacttatatccactgggtccggcaagctccagggaagggcctggagtgggtcgcacgtatttatcccacaaatggttacacacggtatgcggactctgtgaagggccgattcaccatctccgcagacacttccaagaacaccgcgtatctgcaaatgaacagtctgagagctgaggacacggccgtttattactgttcaagatggggcggagacggtttctacgctatggactactggggccaagggaccctggtcaccgtctcctca

SEQ ID NO: 159 - protein, 8 aa, synthetic construct
  REGION 1..8: note = Description of Artificial Sequence: Synthetic peptide
GFNIKDTY

SEQ ID NO: 160 - DNA, 24 bp, synthetic construct
  misc_feature 1..24: note = Description of Artificial Sequence: Synthetic oligonucleotide
  source 1..24: mol_type = other DNA
ggattcaacattaaagatacttat

SEQ ID NO: 161 - protein, 13 aa, synthetic construct
  REGION 1..13: note = Description of Artificial Sequence: Synthetic peptide
SRWGGDGFYAMDY

SEQ ID NO: 162 - DNA, 39 bp, synthetic construct
  misc_feature 1..39: note = Description of Artificial Sequence: Synthetic oligonucleotide
  source 1..39: mol_type = other DNA
tcaagatggggcggagacggtttctacgctatggactac

SEQ ID NO: 163 - protein, 8 aa, synthetic construct
  REGION 1..8: note = Description of Artificial Sequence: Synthetic peptide
IYPTNGYT

SEQ ID NO: 164 - DNA, 24 bp, synthetic construct
  misc_feature 1..24: note = Description of Artificial Sequence: Synthetic oligonucleotide
  source 1..24: mol_type = other DNA
atttatcccacaaatggttacaca

SEQ ID NO: 165 - protein, 110 aa, synthetic construct; identical to SEQ ID NO: 13
  REGION 1..110: note = Description of Artificial Sequence: Synthetic polypeptide

SEQ ID NO: 166 - DNA, 330 bp, synthetic construct; identical to SEQ ID NO: 14
  misc_feature 1..330: note = Description of Artificial Sequence: Synthetic polynucleotide
  source 1..330: mol_type = other DNA

SEQ ID NO: 167 - protein, 106 aa, synthetic construct
  REGION 1..106: note = Description of Artificial Sequence: Synthetic polypeptide
GQPREPQVYTYPPSRDELTKNQVSLTCLVKGFYPSDIAVEWESNGQPENNYKTTPPVLDEDGSFALVSKLTVDKSRWQQGNVFSCSVMHEALHNHYTQKSLSLSPG

SEQ ID NO: 168 - DNA, 318 bp, synthetic construct
  misc_feature 1..318: note = Description of Artificial Sequence: Synthetic polynucleotide
  source 1..318: mol_type = other DNA
ggccagccaagggagccccaggtgtacacatacccacccagcagagacgaactgaccaagaaccaggtgtccctgacatgtctggtgaaaggcttctatcctagtgatattgctgtggagtgggaatcaaatggacagccagagaacaattacaagaccacacctccagtgctggacgaggatggcagcttcgccctggtgtccaagctgacagtggataaatctcgatggcagcaggggaacgtgtttagttgttcagtgatgcatgaagccctgcacaatcattacactcagaagagcctgtccctgtctcccggc

SEQ ID NO: 169 - protein, 481 aa, synthetic construct
  REGION 1..481: note = Description of Artificial Sequence: Synthetic polypeptide
DIQMTQSPSSLSASVGDRVTITCRASQDVNTAVAWYQQKPGKAPKLLIYSASFLYSGVPSRFSGSRSGTDFTLTISSLQPEDFATYYCQQHYTTPPTFGQGTKVEIKGGSGGGSGGGSGGGSGGGSGEVQLVESGGGLVQPGGSLRLSCAASGFNIKDTYIHWVRQAPGKGLEWVARIYPTNGYTRYADSVKGRFTISADTSKNTAYLQMNSLRAEDTAVYYCSRWGGDGFYAMDYWGQGTLVTVSSAAEPKSSDKTHTCPPCPAPELLGGPSVFLFPPKPKDTLMISRTPEVTCVVVDVSHEDPEVKFNWYVDGVEVHNAKTKPREEQYNSTYRVVSVLTVLHQDWLNGKEYKCKVSNKALPAPIEKTISKAKGQPREPQVYTLPPSRDELTKNQVSLICLVKGFYPSDIAVEWESNGQPENRYMTWPPVLDSDGSFFLYSKLTVDKSRWQQGNVFSCSVMHEALHNHYTQKSLSLSPGK

SEQ ID NO: 170 - DNA, 1443 bp, synthetic construct
  misc_feature 1..1443: note = Description of Artificial Sequence: Synthetic polynucleotide
  source 1..1443: mol_type = other DNA
gacatccagatgacccagtctccatcctccctgtctgcatctgtaggagacagagtcaccatcacttgccgggcaagtcaggacgttaacaccgctgtagcttggtatcagcagaaaccagggaaagcccctaagctcctgatctattctgcatcctttttgtacagtggggtcccatcaaggttcagtggcagtcgatctgggacagatttcactctcaccatcagcagtctgcaacctgaagattttgcaacttactactgtcaacagcattacactaccccacccactttcggccaagggaccaaagtggagatcaaaggtggttctggtggtggttctggtggtggttctggtggtggttctggtggtggttctggtgaagtgcagctggtggagtctgggggaggcttggtacagcctggcgggtccctgagactctcctgtgcagcctctggattcaacattaaagatacttatatccactgggtccggcaagctccagggaagggcctggagtgggtcgcacgtatttatcccacaaatggttacacacggtatgcggactctgtgaagggccgattcaccatctccgcagacacttccaagaacaccgcgtatctgcaaatgaacagtctgagagctgaggacacggccgtttattactgttcaagatggggcggagacggtttctacgctatggactactggggccaagggaccctggtcaccgtctcctcagccgccgagcccaagagcagcgataagacccacacctgccctccctgtccagctccagaactgctgggaggacctagcgtgttcctgtttccccctaagccaaaagacactctgatgatttccaggactcccgaggtgacctgcgtggtggtggacgtgtctcacgaggaccccgaagtgaagttcaactggtacgtggatggcgtggaagtgcataatgctaagacaaaaccaagagaggaacagtacaactccacttatcgcgtcgtgagcgtgctgaccgtgctgcaccaggactggctgaacgggaaggagtataagtgcaaagtcagtaataaggccctgcctgctccaatcgaaaaaaccatctctaaggccaaaggccagccaagggagccccaggtgtacacactgccacccagcagagacgaactgaccaagaaccaggtgtccctgatctgtctggtgaaaggcttctatcctagtgatattgctgtggagtgggaatcaaatggacagccagagaacagatacatgacctggcctccagtgctggacagcgatggcagcttcttcctgtattccaagctgacagtggataaatctcgatggcagcaggggaacgtgtttagttgttcagtgatgcatgaagccctgcacaatcattacactcagaagagcctgtccctgtctcccggcaaa

SEQ ID NO: 171 - protein, 107 aa, synthetic construct [sequence omitted]

SEQ ID NO: 172 - DNA, 321 bp, synthetic construct; identical to SEQ ID NO: 150
  misc_feature 1..321: note = Description of Artificial Sequence: Synthetic polynucleotide
  source 1..321: mol_type = other DNA

SEQ ID NO: 173 - protein, 6 aa, synthetic construct
  REGION 1..6: note = Description of Artificial Sequence: Synthetic peptide
QDVNTA

SEQ ID NO: 174 - DNA, 18 bp, synthetic construct
  misc_feature 1..18: note = Description of Artificial Sequence: Synthetic oligonucleotide
  source 1..18: mol_type = other DNA
caggacgttaacaccgct

SEQ ID NO: 175 - protein, 9 aa, synthetic construct
  REGION 1..9: note = Description of Artificial Sequence: Synthetic peptide
QQHYTTPPT

SEQ ID NO: 176 - DNA, 27 bp, synthetic construct
  misc_feature 1..27: note = Description of Artificial Sequence: Synthetic oligonucleotide
  source 1..27: mol_type = other DNA
caacagcattacactaccccacccact

SEQ ID NO: 177-178 - skipped (2 entries)

SEQ ID NO: 179 - protein, 120 aa, synthetic construct [sequence omitted]

SEQ ID NO: 180 - DNA, 360 bp, synthetic construct; identical to SEQ ID NO: 158
  misc_feature 1..360: note = Description of Artificial Sequence: Synthetic polynucleotide
  source 1..360: mol_type = other DNA

SEQ ID NO: 181 - protein, 8 aa, synthetic construct
  REGION 1..8: note = Description of Artificial Sequence: Synthetic peptide
GFNIKDTY

SEQ ID NO: 182 - DNA, 24 bp, synthetic construct
  misc_feature 1..24: note = Description of Artificial Sequence: Synthetic oligonucleotide
  source 1..24: mol_type = other DNA
ggattcaacattaaagatacttat

SEQ ID NO: 183 - protein, 13 aa, synthetic construct
  REGION 1..13: note = Description of Artificial Sequence: Synthetic peptide
SRWGGDGFYAMDY

SEQ ID NO: 184 - DNA, 39 bp, synthetic construct; identical to SEQ ID NO: 162
  misc_feature 1..39: note = Description of Artificial Sequence: Synthetic oligonucleotide
  source 1..39: mol_type = other DNA

SEQ ID NO: 185 - protein, 8 aa, synthetic construct
  REGION 1..8: note = Description of Artificial Sequence: Synthetic peptide
IYPTNGYT

SEQ ID NO: 186 - DNA, 24 bp, synthetic construct
  misc_feature 1..24: note = Description of Artificial Sequence: Synthetic oligonucleotide
  source 1..24: mol_type = other DNA
atttatcccacaaatggttacaca

SEQ ID NO: 187 - protein, 110 aa, synthetic construct; identical to SEQ ID NO: 13
  REGION 1..110: note = Description of Artificial Sequence: Synthetic polypeptide

SEQ ID NO: 188 - DNA, 330 bp, synthetic construct; identical to SEQ ID NO: 14
  misc_feature 1..330: note = Description of Artificial Sequence: Synthetic polynucleotide
  source 1..330: mol_type = other DNA

SEQ ID NO: 189 - protein, 106 aa, synthetic construct; identical to SEQ ID NO: 145
  REGION 1..106: note = Description of Artificial Sequence: Synthetic polypeptide

SEQ ID NO: 190 - DNA, 318 bp, synthetic construct; identical to SEQ ID NO: 146
  misc_feature 1..318: note = Description of Artificial Sequence: Synthetic polynucleotide
  source 1..318: mol_type = other DNA

SEQ ID NO: 191 - protein, 214 aa, synthetic construct
  REGION 1..214: note = Description of Artificial Sequence: Synthetic polypeptide
DIQMTQSPSSLSASVGDRVTITCRASQDVNTAVAWYQQKPGKAPKLLIYSASFLYSGVPSRFSGSRSGTDFTLTISSLQPEDFATYYCQQHYTTPPTFGQGTKVEIKRTVAAPSVFIFPPSDEQLKSGTASVVCLLNNFYPREAKVQWKVDNALQSGNSQESVTEQDSKDSTYSLSSTLTLSKADYEKHKVYACEVTHQGLSSPVTKSFNRGEC

SEQ ID NO: 192 - DNA, 642 bp, synthetic construct
  misc_feature 1..642: note = Description of Artificial Sequence: Synthetic polynucleotide
  source 1..642: mol_type = other DNA
gatattcagatgacccagtcccctagctccctgtccgcttctgtgggcgacagggtcactatcacctgccgcgcatctcaggatgtgaacaccgcagtcgcctggtaccagcagaagcctgggaaagctccaaagctgctgatctacagtgcatcattcctgtattcaggagtgcccagccggtttagcggcagcagatctggcaccgacttcacactgactatctctagtctgcagcctgaggattttgccacatactattgccagcagcactataccacaccccctactttcggccaggggaccaaagtggagatcaagcgaactgtggccgctccaagtgtcttcatttttccacccagcgacgaacagctgaaatccggcacagcttctgtggtctgtctgctgaacaacttctaccccagagaggccaaagtgcagtggaaggtcgataacgctctgcagagtggcaacagccaggagagcgtgacagaacaggactccaaagattctacttatagtctgtcaagcaccctgacactgagcaaggcagactacgaaaagcataaagtgtatgcctgtgaggtgacccatcaggggctgtcttctcccgtgaccaagtctttcaaccgaggcgaatgt

SEQ ID NO: 193 - protein, 107 aa, synthetic construct [sequence omitted]

SEQ ID NO: 194 - DNA, 321 bp, synthetic construct
  misc_feature 1..321: note = Description of Artificial Sequence: Synthetic polynucleotide
  source 1..321: mol_type = other DNA
gatattcagatgacccagtcccctagctccctgtccgcttctgtgggcgacagggtcactatcacctgccgcgcatctcaggatgtgaacaccgcagtcgcctggtaccagcagaagcctgggaaagctccaaagctgctgatctacagtgcatcattcctgtattcaggagtgcccagccggtttagcggcagcagatctggcaccgacttcacactgactatctctagtctgcagcctgaggattttgccacatactattgccagcagcactataccacaccccctactttcggccaggggaccaaagtggagatcaag

SEQ ID NO: 195 - protein, 6 aa, synthetic construct
  REGION 1..6: note = Description of Artificial Sequence: Synthetic peptide
QDVNTA

SEQ ID NO: 196 - DNA, 18 bp, synthetic construct
  misc_feature 1..18: note = Description of Artificial Sequence: Synthetic oligonucleotide
  source 1..18: mol_type = other DNA
caggatgtgaacaccgca

SEQ ID NO: 197 - protein, 9 aa, synthetic construct
  REGION 1..9: note = Description of Artificial Sequence: Synthetic peptide
QQHYTTPPT

SEQ ID NO: 198 - DNA, 27 bp, synthetic construct
  misc_feature 1..27: note = Description of Artificial Sequence: Synthetic oligonucleotide
  source 1..27: mol_type = other DNA
cagcagcactataccacaccccctact

SEQ ID NO: 199-200 - skipped (2 entries)

SEQ ID NO: 201 - protein, 107 aa, synthetic construct [sequence omitted]

SEQ ID NO: 202 - DNA, 321 bp, synthetic construct
  misc_feature 1..321: note = Description of Artificial Sequence: Synthetic polynucleotide
  source 1..321: mol_type = other DNA
cgaactgtggccgctccaagtgtcttcatttttccacccagcgacgaacagctgaaatccggcacagcttctgtggtctgtctgctgaacaacttctaccccagagaggccaaagtgcagtggaaggtcgataacgctctgcagagtggcaacagccaggagagcgtgacagaacaggactccaaagattctacttatagtctgtcaagcaccctgacactgagcaaggcagactacgaaaagcataaagtgtatgcctgtgaggtgacccatcaggggctgtcttctcccgtgaccaagtctttcaaccgaggcgaatgt

SEQ ID NO: 203 - protein, 448 aa, synthetic construct
  REGION 1..448: note = Description of Artificial Sequence: Synthetic polypeptide
EVQLVESGGGLVQPGGSLRLSCAASGFTFTDYTMDWVRQAPGKGLEWVADVNPNSGGSIYNQRFKGRFTLSVDRSKNTLYLQMNSLRAEDTAVYYCARNLGPSFYFDYWGQGTLVTVSSASTKGPSVFPLAPSSKSTSGGTAALGCLVKDYFPEPVTVSWNSGALTSGVHTFPAVLQSSGLYSLSSVVTVPSSSLGTQTYICNVNHKPSNTKVDKKVEPKSCDKTHTCPPCPAPELLGGPSVFLFPPKPKDTLMISRTPEVTCVVVDVSHEDPEVKFNWYVDGVEVHNAKTKPREEQYNSTYRVVSVLTVLHQDWLNGKEYKCKVSNKALPAPIEKTISKAKGQPREPQVYVLPPSRDELTKNQVSLLCLVKGFYPSDIAVEWESNGQPENNYLTWPPVLDSDGSFFLYSKLTVDKSRWQQGNVFSCSVMHEALHNHYTQKSLSLSPG

SEQ ID NO: 204 - DNA, 1344 bp, synthetic construct
  misc_feature 1..1344: note = Description of Artificial Sequence: Synthetic polynucleotide
  source 1..1344: mol_type = other DNA
gaagtgcagctggtcgaatctggaggaggactggtgcagccaggagggtccctgcgcctgtcttgcgccgctagtggcttcacttttaccgactacaccatggattgggtgcgacaggcacctggaaagggcctggagtgggtcgccgatgtgaacccaaatagcggaggctccatctacaaccagcggttcaagggccggttcaccctgtcagtggaccggagcaaaaacaccctgtatctgcagatgaatagcctgcgagccgaagatactgctgtgtactattgcgcccggaatctggggccctccttctactttgactattgggggcagggaactctggtcaccgtgagctccgcctccaccaagggaccttctgtgttcccactggctccctctagtaaatccacatctgggggaactgcagccctgggctgtctggtgaaggactacttcccagagcccgtcacagtgtcttggaacagtggcgctctgacttctggggtccacacctttcctgcagtgctgcagtcaagcgggctgtacagcctgtcctctgtggtcaccgtgccaagttcaagcctgggaacacagacttatatctgcaacgtgaatcacaagccatccaatacaaaagtcgacaagaaagtggaacccaagtcttgtgataaaacccatacatgccccccttgtcctgcaccagagctgctgggaggaccaagcgtgttcctgtttccacccaagcctaaagatacactgatgattagtaggaccccagaagtcacatgcgtggtcgtggacgtgagccacgaggaccccgaagtcaagtttaactggtacgtggacggcgtcgaggtgcataatgccaagactaaacccagggaggaacagtacaacagtacctatcgcgtcgtgtcagtcctgacagtgctgcatcaggattggctgaacgggaaagagtataagtgcaaagtgagcaataaggctctgcccgcacctatcgagaaaacaatttccaaggcaaaaggacagcctagagaaccacaggtgtacgtgctgcctccatcaagggatgagctgacaaagaaccaggtcagcctgctgtgtctggtgaaaggattctatccctctgacattgctgtggagtgggaaagtaatggccagcctgagaacaattacctgacctggccccctgtgctggactcagatggcagcttctttctgtatagcaagctgaccgtcgacaaatcccggtggcagcaggggaatgtgtttagttgttcagtcatgcacgaggcactgcacaaccattacacccagaagtcactgtcactgtcaccaggg

SEQ ID NO: 205 - protein, 119 aa, synthetic construct [sequence omitted]

SEQ ID NO: 206 - DNA, 357 bp, synthetic construct; identical to SEQ ID NO: 20
  misc_feature 1..357: note = Description of Artificial Sequence: Synthetic polynucleotide
  source 1..357: mol_type = other DNA

SEQ ID NO: 207 - protein, 8 aa, synthetic construct
  REGION 1..8: note = Description of Artificial Sequence: Synthetic peptide
GFTFTDYT

SEQ ID NO: 208 - DNA, 24 bp, synthetic construct
  misc_feature 1..24: note = Description of Artificial Sequence: Synthetic oligonucleotide
  source 1..24: mol_type = other DNA
ggcttcacttttaccgactacacc

SEQ ID NO: 209 - protein, 12 aa, synthetic construct
  REGION 1..12: note = Description of Artificial Sequence: Synthetic peptide
ARNLGPSFYFDY

SEQ ID NO: 210 - DNA, 36 bp, synthetic construct; identical to SEQ ID NO: 24
  misc_feature 1..36: note = Description of Artificial Sequence: Synthetic oligonucleotide
  source 1..36: mol_type = other DNA

SEQ ID NO: 211 - protein, 8 aa, synthetic construct
  REGION 1..8: note = Description of Artificial Sequence: Synthetic peptide
VNPNSGGS

SEQ ID NO: 212 - DNA, 24 bp, synthetic construct
  misc_feature 1..24: note = Description of Artificial Sequence: Synthetic oligonucleotide
  source 1..24: mol_type = other DNA
gtgaacccaaatagcggaggctcc

SEQ ID NO: 213 - protein, 98 aa, synthetic construct; identical to SEQ ID NO: 11
  REGION 1..98: note = Description of Artificial Sequence: Synthetic polypeptide

SEQ ID NO: 214 - DNA, 294 bp, synthetic construct
  misc_feature 1..294: note = Description of Artificial Sequence: Synthetic polynucleotide
  source 1..294: mol_type = other DNA
gcctccaccaagggaccttctgtgttcccactggctccctctagtaaatccacatctgggggaactgcagccctgggctgtctggtgaaggactacttcccagagcccgtcacagtgtcttggaacagtggcgctctgacttctggggtccacacctttcctgcagtgctgcagtcaagcgggctgtacagcctgtcctctgtggtcaccgtgccaagttcaagcctgggaacacagacttatatctgcaacgtgaatcacaagccatccaatacaaaagtcgacaagaaagtg

SEQ ID NO: 215 - protein, 110 aa, synthetic construct; identical to SEQ ID NO: 13
  REGION 1..110: note = Description of Artificial Sequence: Synthetic polypeptide

SEQ ID NO: 216 - DNA, 330 bp, synthetic construct; identical to SEQ ID NO: 30
  misc_feature 1..330: note = Description of Artificial Sequence: Synthetic polynucleotide
  source 1..330: mol_type = other DNA

SEQ ID NO: 217 - protein, 106 aa, synthetic construct; identical to SEQ ID NO: 31
  REGION 1..106: note = Description of Artificial Sequence: Synthetic polypeptide

SEQ ID NO: 218 - DNA, 318 bp, synthetic construct; identical to SEQ ID NO: 32
  misc_feature 1..318: note = Description of Artificial Sequence: Synthetic polynucleotide
  source 1..318: mol_type = other DNA

SEQ ID NO: 219 - protein, 448 aa, synthetic construct
  REGION 1..448: note = Description of Artificial Sequence: Synthetic polypeptide
EVQLVESGGGLVQPGGSLRLSCAASGFTFTDYTMDWVRQAPGKGLEWVADVNPNSGGSIYNQRFKGRFTLSVDRSKNTLYLQMNSLRAEDTAVYYCARNLGPSFYFDYWGQGTLVTVSSASTKGPSVFPLAPSSKSTSGGTAALGCLVKDYFPEPVTVSWNSGALTSGVHTFPAVLQSSGLYSLSSVVTVPSSSLGTQTYICNVNHKPSNTKVDKKVEPKSCDKTHTCPPCPAPELLGGPSVFLFPPKPKDTLMISRTPEVTCVVVDVSHEDPEVKFNWYVDGVEVHNAKTKPREEQYNSTYRVVSVLTVLHQDWLNGKEYKCKVSNKALPAPIEKTISKAKGQPREPQVYVYPPSRDELTKNQVSLTCLVKGFYPSDIAVEWESNGQPENNYKTTPPVLDSDGSFALVSKLTVDKSRWQQGNVFSCSVMHEALHNHYTQKSLSLSPG

SEQ ID NO: 220 - DNA, 1344 bp, synthetic construct
  misc_feature 1..1344: note = Description of Artificial Sequence: Synthetic polynucleotide
  source 1..1344: mol_type = other DNA
gaagtgcagctggtcgaatctggaggaggactggtgcagccaggagggtccctgcgcctgtcttgcgccgctagtggcttcacttttaccgactacaccatggattgggtgcgacaggcacctggaaagggcctggagtgggtcgccgatgtgaacccaaatagcggaggctccatctacaaccagcggttcaagggccggttcaccctgtcagtggaccggagcaaaaacaccctgtatctgcagatgaatagcctgcgagccgaagatactgctgtgtactattgcgcccggaatctggggccctccttctactttgactattgggggcagggaactctggtcaccgtgagctccgcctccaccaagggaccttctgtgttcccactggctccctctagtaaatccacatctgggggaactgcagccctgggctgtctggtgaaggactacttcccagagcccgtcacagtgtcttggaacagtggcgctctgacttctggggtccacacctttcctgcagtgctgcagtcaagcgggctgtacagcctgtcctctgtggtcaccgtgccaagttcaagcctgggaacacagacttatatctgcaacgtgaatcacaagccatccaatacaaaagtcgacaagaaagtggaacccaagtcttgtgataaaacccatacatgccccccttgtcctgcaccagagctgctgggaggaccaagcgtgttcctgtttccacccaagcctaaagatacactgatgattagtaggaccccagaagtcacatgcgtggtcgtggacgtgagccacgaggaccccgaagtcaagtttaactggtacgtggacggcgtcgaggtgcataatgccaagactaaacccagggaggaacagtacaacagtacctatcgcgtcgtgtcagtcctgacagtgctgcatcaggattggctgaacgggaaagagtataagtgcaaagtgagcaataaggctctgcccgcacctatcgagaaaacaatttccaaggcaaaaggacagcctagagaaccacaggtgtacgtgtatcctccatcaagggatgagctgacaaagaaccaggtcagcctgacttgtctggtgaaaggattctatccctctgacattgctgtggagtgggaaagtaatggccagcctgagaacaattacaagaccacaccccctgtgctggactcagatggcagcttcgcgctggtgagcaagctgaccgtcgacaaatcccggtggcagcaggggaatgtgtttagttgttcagtcatgcacgaggcactgcacaaccattacacccagaagtcactgtcactgtcaccaggg

SEQ ID NO: 221 - protein, 119 aa, synthetic construct [sequence omitted]

SEQ ID NO: 222 - DNA, 357 bp, synthetic construct; identical to SEQ ID NO: 20
  misc_feature 1..357: note = Description of Artificial Sequence: Synthetic polynucleotide
  source 1..357: mol_type = other DNA

SEQ ID NO: 223 - protein, 8 aa, synthetic construct
  REGION 1..8: note = Description of Artificial Sequence: Synthetic peptide
GFTFTDYT

SEQ ID NO: 224 - DNA, 24 bp, synthetic construct
  misc_feature 1..24: note = Description of Artificial Sequence: Synthetic oligonucleotide
  source 1..24: mol_type = other DNA
ggcttcacttttaccgactacacc

SEQ ID NO: 225 - protein, 12 aa, synthetic construct
  REGION 1..12: note = Description of Artificial Sequence: Synthetic peptide
ARNLGPSFYFDY

SEQ ID NO: 226 - DNA, 36 bp, synthetic construct; identical to SEQ ID NO: 24
  misc_feature 1..36: note = Description of Artificial Sequence: Synthetic oligonucleotide
  source 1..36: mol_type = other DNA

SEQ ID NO: 227 - protein, 8 aa, synthetic construct
  REGION 1..8: note = Description of Artificial Sequence: Synthetic peptide
VNPNSGGS

SEQ ID NO: 228 - DNA, 24 bp, synthetic construct
  misc_feature 1..24: note = Description of Artificial Sequence: Synthetic oligonucleotide
  source 1..24: mol_type = other DNA
gtgaacccaaatagcggaggctcc

SEQ ID NO: 229 - protein, 98 aa, synthetic construct; identical to SEQ ID NO: 11
  REGION 1..98: note = Description of Artificial Sequence: Synthetic polypeptide

SEQ ID NO: 230 - DNA, 294 bp, synthetic construct; identical to SEQ ID NO: 214
  misc_feature 1..294: note = Description of Artificial Sequence: Synthetic polynucleotide
  source 1..294: mol_type = other DNA

SEQ ID NO: 231 - protein, 110 aa, synthetic construct; identical to SEQ ID NO: 13
  REGION 1..110: note = Description of Artificial Sequence: Synthetic polypeptide

SEQ ID NO: 232 - DNA, 330 bp, synthetic construct; identical to SEQ ID NO: 30
  misc_feature 1..330: note = Description of Artificial Sequence: Synthetic polynucleotide
  source 1..330: mol_type = other DNA

SEQ ID NO: 233 - protein, 106 aa, synthetic construct; identical to SEQ ID NO: 95
  REGION 1..106: note = Description of Artificial Sequence: Synthetic polypeptide

SEQ ID NO: 234 - DNA, 318 bp, synthetic construct
  misc_feature 1..318: note = Description of Artificial Sequence: Synthetic polynucleotide
  source 1..318: mol_type = other DNA
ggacagcctagagaaccacaggtgtacgtgtatcctccatcaagggatgagctgacaaagaaccaggtcagcctgacttgtctggtgaaaggattctatccctctgacattgctgtggagtgggaaagtaatggccagcctgagaacaattacaagaccacaccccctgtgctggactcagatggcagcttcgcgctggtgagcaagctgaccgtcgacaaatcccggtggcagcaggggaatgtgtttagttgttcagtcatgcacgaggcactgcacaaccattacacccagaagtcactgtcactgtcaccaggg

SEQ ID NO: 235 - protein, 450 aa, synthetic construct; identical to SEQ ID NO: 125
  REGION 1..450: note = Description of Artificial Sequence: Synthetic polypeptide

SEQ ID NO: 236 - DNA, 1350 bp, synthetic construct
  misc_feature 1..1350: note = Description of Artificial Sequence: Synthetic polynucleotide
  source 1..1350: mol_type = other DNA
gaggtgcagctggtggaaagcggaggaggactggtgcagccaggaggatctctgcgactgagttgcgccgcttcaggattcaacatcaaggacacctacattcactgggtgcgacaggctccaggaaaaggactggagtgggtggctcgaatctatcccactaatggatacacccggtatgccgactccgtgaaggggaggtttactattagcgccgatacatccaaaaacactgcttacctgcagatgaacagcctgcgagccgaagataccgctgtgtactattgcagtcgatggggaggagacggattctacgctatggattattggggacaggggaccctggtgacagtgagctccgcctctaccaagggccccagtgtgtttcccctggctccttctagtaaatccacctctggagggacagccgctctgggatgtctggtgaaggactatttccccgagcctgtgaccgtgagttggaactcaggcgccctgacaagcggagtgcacacttttcctgctgtgctgcagtcaagcgggctgtactccctgtcctctgtggtgacagtgccaagttcaagcctgggcacacagacttatatctgcaacgtgaatcataagccctcaaatacaaaagtggacaagaaagtggagcccaagagctgtgataagacccacacctgccctccctgtccagctccagaactgctgggaggacctagcgtgttcctgtttccccctaagccaaaagacactctgatgatttccaggactcccgaggtgacctgcgtggtggtggacgtgtctcacgaggaccccgaagtgaagttcaactggtacgtggatggcgtggaagtgcataatgctaagacaaaaccaagagaggaacagtacaactccacttatcgcgtcgtgagcgtgctgaccgtgctgcaccaggactggctgaacgggaaggagtataagtgcaaagtcagtaataaggccctgcctgctccaatcgaaaaaaccatctctaaggccaaaggccagccaagggagccccaggtgtacgtgtacccacccagcagagacgaactgaccaagaaccaggtgtccctgacatgtctggtgaaaggcttctatcctagtgatattgctgtggagtgggaatcaaatggacagccagagaacaattacaagaccacacctccagtgctggacagcgatggcagcttcgccctggtgtccaagctgacagtggataaatctcgatggcagcaggggaacgtgtttagttgttcagtgatgcatgaagccctgcacaatcattacactcagaagagcctgtccctgtctcccggcaaa

SEQ ID NO: 237 - protein, 120 aa, synthetic construct [sequence omitted]

SEQ ID NO: 238 - DNA, 360 bp, synthetic construct; identical to SEQ ID NO: 4
  misc_feature 1..360: note = Description of Artificial Sequence: Synthetic polynucleotide
  source 1..360: mol_type = other DNA

SEQ ID NO: 239 - protein, 8 aa, synthetic construct
  REGION 1..8: note = Description of Artificial Sequence: Synthetic peptide
GFNIKDTY

SEQ ID NO: 240 - DNA, 24 bp, synthetic construct
  misc_feature 1..24: note = Description of Artificial Sequence: Synthetic oligonucleotide
  source 1..24: mol_type = other DNA
ggattcaacatcaaggacacctac

SEQ ID NO: 241 - protein, 13 aa, synthetic construct
  REGION 1..13: note = Description of Artificial Sequence: Synthetic peptide
SRWGGDGFYAMDY

SEQ ID NO: 242 - DNA, 39 bp, synthetic construct; identical to SEQ ID NO: 8
  misc_feature 1..39: note = Description of Artificial Sequence: Synthetic oligonucleotide
  source 1..39: mol_type = other DNA

SEQ ID NO: 243 - protein, 8 aa, synthetic construct
  REGION 1..8: note = Description of Artificial Sequence: Synthetic peptide
IYPTNGYT

SEQ ID NO: 244 - DNA, 24 bp, synthetic construct
  misc_feature 1..24: note = Description of Artificial Sequence: Synthetic oligonucleotide
  source 1..24: mol_type = other DNA
atctatcccactaatggatacacc

SEQ ID NO: 245 - protein, 98 aa, synthetic construct; identical to SEQ ID NO: 11
  REGION 1..98: note = Description of Artificial Sequence: Synthetic polypeptide

SEQ ID NO: 246 - DNA, 294 bp, synthetic construct; identical to SEQ ID NO: 12
  misc_feature 1..294: note = Description of Artificial Sequence: Synthetic polynucleotide
  source 1..294: mol_type = other DNA

SEQ ID NO: 247 - protein, 110 aa, synthetic construct; identical to SEQ ID NO: 13
  REGION 1..110: note = Description of Artificial Sequence: Synthetic polypeptide

SEQ ID NO: 248 - DNA, 330 bp, synthetic construct; identical to SEQ ID NO: 14
  misc_feature 1..330: note = Description of Artificial Sequence: Synthetic polynucleotide
  source 1..330: mol_type = other DNA

SEQ ID NO: 249 - protein, 106 aa, synthetic construct; identical to SEQ ID NO: 95
  REGION 1..106: note = Description of Artificial Sequence: Synthetic polypeptide

SEQ ID NO: 250 - DNA, 318 bp, synthetic construct
  misc_feature 1..318: note = Description of Artificial Sequence: Synthetic polynucleotide
  source 1..318: mol_type = other DNA
ggccagccaagggagccccaggtgtacgtgtacccacccagcagagacgaactgaccaagaaccaggtgtccctgacatgtctggtgaaaggcttctatcctagtgatattgctgtggagtgggaatcaaatggacagccagagaacaattacaagaccacacctccagtgctggacagcgatggcagcttcgccctggtgtccaagctgacagtggataaatctcgatggcagcaggggaacgtgtttagttgttcagtgatgcatgaagccctgcacaatcattacactcagaagagcctgtccctgtctcccggc

SEQ ID NO: 251 - protein, 232 aa, synthetic construct
  REGION 1..232: note = Description of Artificial Sequence: Synthetic polypeptide
EPKSSDKTHTCPPCPAPELLGGPSVFLFPPKPKDTLMISRTPEVTCVVVDVSHEDPEVKFNWYVDGVEVHNAKTKPREEQYNSTYRVVSVLTVLHQDWLNGKEYKCKVSNKALPAPIEKTISKAKGQPREPQVYVLPPSRDELTKNQVSLLCLVKGFYPSDIAVEWESNGQPENNYLTWPPVLDSDGSFFLYSKLTVDKSRWQQGNVFSCSVMHEALHNHYTQKSLSLSPGK

SEQ ID NO: 252 - DNA, 696 bp, synthetic construct
  misc_feature 1..696: note = Description of Artificial Sequence: Synthetic polynucleotide
  source 1..696: mol_type = other DNA
gaacctaaaagcagcgacaagacccacacatgccccccttgtccagctccagaactgctgggaggaccaagcgtgttcctgtttccacccaagcccaaagatacactgatgatcagccgaactcccgaggtcacctgcgtggtcgtggacgtgtcccacgaggaccccgaagtcaagttcaactggtacgtggacggcgtcgaagtgcataatgcaaagactaaaccacgggaggaacagtacaactctacatatagagtcgtgagtgtcctgactgtgctgcatcaggattggctgaacggcaaagagtataagtgcaaagtgtctaataaggccctgcctgctccaatcgagaaaactattagtaaggcaaaagggcagcccagggaacctcaggtctacgtgctgcctccaagtcgcgacgagctgaccaagaaccaggtctcactgctgtgtctggtgaaaggattctatccttccgatattgccgtggagtgggaatctaatggccagccagagaacaattacctgacctggccccctgtgctggacagcgatgggtccttctttctgtattcaaagctgacagtggacaaaagcagatggcagcagggaaacgtctttagctgttccgtgatgcacgaagccctgcacaatcattacacccagaagtctctgagtctgtcacctggcaaa

SEQ ID NO: 253 - protein, 110 aa, synthetic construct; identical to SEQ ID NO: 13
  REGION 1..110: note = Description of Artificial Sequence: Synthetic polypeptide

SEQ ID NO: 254 - DNA, 330 bp, synthetic construct
  misc_feature 1..330: note = Description of Artificial Sequence: Synthetic polynucleotide
  source 1..330: mol_type = other DNA
gctccagaactgctgggaggaccaagcgtgttcctgtttccacccaagcccaaagatacactgatgatcagccgaactcccgaggtcacctgcgtggtcgtggacgtgtcccacgaggaccccgaagtcaagttcaactggtacgtggacggcgtcgaagtgcataatgcaaagactaaaccacgggaggaacagtacaactctacatatagagtcgtgagtgtcctgactgtgctgcatcaggattggctgaacggcaaagagtataagtgcaaagtgtctaataaggccctgcctgctccaatcgagaaaactattagtaaggcaaaa

SEQ ID NO: 255 - protein, 106 aa, synthetic construct; identical to SEQ ID NO: 31
  REGION 1..106: note = Description of Artificial Sequence: Synthetic polypeptide

SEQ ID NO: 256 - DNA, 318 bp, synthetic construct
  misc_feature 1..318: note = Description of Artificial Sequence: Synthetic polynucleotide
  source 1..318: mol_type = other DNA
gggcagcccagggaacctcaggtctacgtgctgcctccaagtcgcgacgagctgaccaagaaccaggtctcactgctgtgtctggtgaaaggattctatccttccgatattgccgtggagtgggaatctaatggccagccagagaacaattacctgacctggccccctgtgctggacagcgatgggtccttctttctgtattcaaagctgacagtggacaaaagcagatggcagcagggaaacgtctttagctgttccgtgatgcacgaagccctgcacaatcattacacccagaagtctctgagtctgtcacctggc

SEQ ID NO: 257 - protein, 475 aa, synthetic construct
  REGION 1..475: note = Description of Artificial Sequence: Synthetic polypeptide
DIQMTQSPSSLSASVGDRVTITCKASQDVSIGVAWYQQKPGKAPKLLIYSASYRYTGVPSRFSGSGSGTDFTLTISSLQPEDFATYYCQQYYIYPYTFGQGTKVEIKGGGGSGGGGSGGGGSEVQLVESGGGLVQPGGSLRLSCAASGFTFTDYTMDWVRQAPGKGLEWVADVNPNSGGSIYNQRFKGRFTLSVDRSKNTLYLQMNSLRAEDTAVYYCARNLGPSFYFDYWGQGTLVTVSSAAEPKSSDKTHTCPPCPAPELLGGPSVFLFPPKPKDTLMISRTPEVTCVVVDVSHEDPEVKFNWYVDGVEVHNAKTKPREEQYNSTYRVVSVLTVLHQDWLNGKEYKCKVSNKALPAPIEKTISKAKGQPREPQVYVYPPSRDELTKNQVSLTCLVKGFYPSDIAVEWESNGQPENNYKTTPPVLDSDGSFALVSKLTVDKSRWQQGNVFSCSVMHEALHNHYTQKSLSLSPGK

SEQ ID NO: 258 - DNA, 1425 bp, synthetic construct
  misc_feature 1..1425: note = Description of Artificial Sequence: Synthetic polynucleotide
  source 1..1425: mol_type = other DNA
gacattcagatgacccagagccctagctccctgagtgcctcagtcggggacagggtgactatcacctgcaaggcttcacaggatgtcagcattggcgtggcatggtaccagcagaagccagggaaagcacccaagctgctgatctatagcgcctcctacaggtatacaggcgtgccatcccgcttctctggcagtgggtcaggaactgactttacactgactatttctagtctgcagcccgaagatttcgccacatactattgccagcagtactatatctacccttatacttttggccaggggaccaaagtggagattaagggcggaggaggctccggaggaggagggtctggaggaggaggaagtgaggtccagctggtggaatctggaggaggactggtgcagccaggagggtccctgaggctgtcttgtgccgctagtggcttcacctttacagactacacaatggattgggtgcgccaggcaccaggaaagggactggaatgggtcgctgatgtgaaccctaatagcggaggctccatctacaaccagcggttcaaaggacggttcaccctgtcagtggaccggagcaagaacaccctgtatctgcagatgaacagcctgagagccgaggatactgctgtgtactattgcgccaggaatctgggcccaagcttctactttgactattgggggcagggaacactggtcactgtgtcaagcgcagccgaacccaaatcctctgataagactcacacctgcccaccttgtccagctccagagctgctgggaggacctagcgtgttcctgtttccacccaagccaaaagacactctgatgatttctagaacccctgaagtgacatgtgtggtcgtggacgtcagtcacgaggaccccgaagtcaaattcaactggtacgtggatggcgtcgaggtgcataatgccaagaccaaaccccgagaggaacagtacaactcaacctatcgggtcgtgagcgtcctgacagtgctgcatcaggactggctgaacggcaaggagtataagtgcaaagtgagcaacaaggctctgcctgcaccaatcgagaagaccatttccaaggctaaagggcagccccgcgaacctcaggtctacgtgtatcctccaagccgagatgagctgacaaaaaaccaggtctccctgacttgtctggtgaagggattttacccaagtgacatcgcagtggagtgggaatcaaatggccagcccgaaaacaattataagaccacaccccctgtgctggactctgatgggagtttcgcactggtctccaaactgaccgtggacaagtctcggtggcagcagggaaacgtctttagctgttccgtgatgcacgaggccctgcacaatcattacacacagaaatctctgagtctgtcacctggcaag

SEQ ID NO: 259 - protein, 107 aa, synthetic construct [sequence omitted]

SEQ ID NO: 260 - DNA, 321 bp, synthetic construct
  misc_feature 1..321: note = Description of Artificial Sequence: Synthetic polynucleotide
  source 1..321: mol_type = other DNA
gacattcagatgacccagagccctagctccctgagtgcctcagtcggggacagggtgactatcacctgcaaggcttcacaggatgtcagcattggcgtggcatggtaccagcagaagccagggaaagcacccaagctgctgatctatagcgcctcctacaggtatacaggcgtgccatcccgcttctctggcagtgggtcaggaactgactttacactgactatttctagtctgcagcccgaagatttcgccacatactattgccagcagtactatatctacccttatacttttggccaggggaccaaagtggagattaag

SEQ ID NO: 261 - protein, 6 aa, synthetic construct
  REGION 1..6: note = Description of Artificial Sequence: Synthetic peptide
QDVSIG

SEQ ID NO: 262 - DNA, 18 bp, synthetic construct
  misc_feature 1..18: note = Description of Artificial Sequence: Synthetic oligonucleotide
  source 1..18: mol_type = other DNA
caggatgtcagcattggc

SEQ ID NO: 263 - protein, 9 aa, synthetic construct
  REGION 1..9: note = Description of Artificial Sequence: Synthetic peptide
QQYYIYPYT

SEQ ID NO: 264 - DNA, 27 bp, synthetic construct
  misc_feature 1..27: note = Description of Artificial Sequence: Synthetic oligonucleotide
  source 1..27: mol_type = other DNA
cagcagtactatatctacccttatact

SEQ ID NO: 265-266 - skipped (2 entries)

SEQ ID NO: 267 - protein, 119 aa, synthetic construct [sequence omitted]

SEQ ID NO: 268 - DNA, 357 bp, synthetic construct
  misc_feature 1..357: note = Description of Artificial Sequence: Synthetic polynucleotide
  source 1..357: mol_type = other DNA
gaggtccagctggtggaatctggaggaggactggtgcagccaggagggtccctgaggctgtcttgtgccgctagtggcttcacctttacagactacacaatggattgggtgcgccaggcaccaggaaagggactggaatgggtcgctgatgtgaaccctaatagcggaggctccatctacaaccagcggttcaaaggacggttcaccctgtcagtggaccggagcaagaacaccctgtatctgcagatgaacagcctgagagccgaggatactgctgtgtactattgcgccaggaatctgggcccaagcttctactttgactattgggggcagggaacactggtcactgtgtcaagc

SEQ ID NO: 269 - protein, 8 aa, synthetic construct
  REGION 1..8: note = Description of Artificial Sequence: Synthetic peptide
GFTFTDYT

SEQ ID NO: 270 - DNA, 24 bp, synthetic construct
  misc_feature 1..24: note = Description of Artificial Sequence: Synthetic oligonucleotide
  source 1..24: mol_type = other DNA
ggcttcacctttacagactacaca

SEQ ID NO: 271 - protein, 12 aa, synthetic construct
  REGION 1..12: note = Description of Artificial Sequence: Synthetic peptide
ARNLGPSFYFDY

SEQ ID NO: 272 - DNA, 36 bp, synthetic construct
  misc_feature 1..36: note = Description of Artificial Sequence: Synthetic oligonucleotide
  source 1..36: mol_type = other DNA
gccaggaatctgggcccaagcttctactttgactat

SEQ ID NO: 273 - protein, 8 aa, synthetic construct
  REGION 1..8: note = Description of Artificial Sequence: Synthetic peptide
VNPNSGGS

SEQ ID NO: 274 - DNA, 24 bp, synthetic construct
  misc_feature 1..24: note = Description of Artificial Sequence: Synthetic oligonucleotide
  source 1..24: mol_type = other DNA
gtgaaccctaatagcggaggctcc

SEQ ID NO: 275 - protein, 110 aa, synthetic construct; identical to SEQ ID NO: 13
  REGION 1..110: note = Description of Artificial Sequence: Synthetic polypeptide

SEQ ID NO: 276 - DNA, 330 bp, synthetic construct
  misc_feature 1..330: note = Description of Artificial Sequence: Synthetic polynucleotide
  source 1..330: mol_type = other DNA
gctccagagctgctgggaggacctagcgtgttcctgtttccacccaagccaaaagacactctgatgatttctagaacccctgaagtgacatgtgtggtcgtggacgtcagtcacgaggaccccgaagtcaaattcaactggtacgtggatggcgtcgaggtgcataatgccaagaccaaaccccgagaggaacagtacaactcaacctatcgggtcgtgagcgtcctgacagtgctgcatcaggactggctgaacggcaaggagtataagtgcaaagtgagcaacaaggctctgcctgcaccaatcgagaagaccatttccaaggctaaa

SEQ ID NO: 277 - protein, 106 aa, synthetic construct; identical to SEQ ID NO: 95
  REGION 1..106: note = Description of Artificial Sequence: Synthetic polypeptide

SEQ ID NO: 278 - DNA, 318 bp, synthetic construct
  misc_feature 1..318: note = Description of Artificial Sequence: Synthetic polynucleotide
  source 1..318: mol_type = other DNA
gggcagccccgcgaacctcaggtctacgtgtatcctccaagccgagatgagctgacaaaaaaccaggtctccctgacttgtctggtgaagggattttacccaagtgacatcgcagtggagtgggaatcaaatggccagcccgaaaacaattataagaccacaccccctgtgctggactctgatgggagtttcgcactggtctccaaactgaccgtggacaagtctcggtggcagcagggaaacgtctttagctgttccgtgatgcacgaggccctgcacaatcattacacacagaaatctctgagtctgtcacctggc

SEQ ID NO: 279 - protein, 450 aa, synthetic construct
  REGION 1..450: note = Description of Artificial Sequence: Synthetic polypeptide
EVQLVESGGGLVQPGGSLRLSCAASGFNIKDTYIHWVRQAPGKGLEWVARIYPTNGYTRYADSVKGRFTISADTSKNTAYLQMNSLRAEDTAVYYCSRWGGDGFYAMDYWGQGTLVTVSSASTKGPSVFPLAPSSKSTSGGTAALGCLVKDYFPEPVTVSWNSGALTSGVHTFPAVLQSSGLYSLSSVVTVPSSSLGTQTYICNVNHKPSNTKVDKKVEPKSCDKTHTCPPCPAPELLGGPSVFLFPPKPKDTLMISRTPEVTCVVVDVSHEDPEVKFNWYVDGVEVHNAKTKPREEQYNSTYRVVSVLTVLHQDWLNGKEYKCKVSNKALPAPIEKTISKAKGQPREPQVYVLPPSRDELTKNQVSLLCLVKGFYPSDIAVEWESNGQPENNYLTWPPVLDSDGSFFLYSKLTVDKSRWQQGNVFSCSVMHEALHNHYTQKSLSLSPGK

SEQ ID NO: 280 - DNA, 1350 bp, synthetic construct
  misc_feature 1..1350: note = Description of Artificial Sequence: Synthetic polynucleotide
  source 1..1350: mol_type = other DNA
gaggtgcagctggtggaaagcggaggaggactggtgcagccaggaggatctctgcgactgagttgcgccgcttcaggattcaacatcaaggacacctacattcactgggtgcgacaggctccaggaaaaggactggagtgggtggctcgaatctatcccactaatggatacacccggtatgccgactccgtgaaggggaggtttactattagcgccgatacatccaaaaacactgcttacctgcagatgaacagcctgcgagccgaagataccgctgtgtactattgcagtcgatggggaggagacggattctacgctatggattattggggacaggggaccctggtgacagtgagctccgcctctaccaagggccccagtgtgtttcccctggctccttctagtaaatccacctctggagggacagccgctctgggatgtctggtgaaggactatttccccgagcctgtgaccgtgagttggaactcaggcgccctgacaagcggagtgcacacttttcctgctgtgctgcagtcaagcgggctgtactccctgtcctctgtggtgacagtgccaagttcaagcctgggcacacagacttatatctgcaacgtgaatcataagccctcaaatacaaaagtggacaagaaagtggagcccaagagctgtgataagacccacacctgccctccctgtccagctccagaactgctgggaggacctagcgtgttcctgtttccccctaagccaaaagacactctgatgatttccaggactcccgaggtgacctgcgtggtggtggacgtgtctcacgaggaccccgaagtgaagttcaactggtacgtggatggcgtggaagtgcataatgctaagacaaaaccaagagaggaacagtacaactccacttatcgcgtcgtgagcgtgctgaccgtgctgcaccaggactggctgaacgggaaggagtataagtgcaaagtcagtaataaggccctgcctgctccaatcgaaaaaaccatctctaaggccaaaggccagccaagggagccccaggtgtacgtgctgccacccagcagagacgaactgaccaagaaccaggtgtccctgctgtgtctggtgaaaggcttctatcctagtgatattgctgtggagtgggaatcaaatggacagccagagaacaattacctgacctggcctccagtgctggacagcgatggcagcttcttcctgtattccaagctgacagtggataaatctcgatggcagcaggggaacgtgtttagttgttcagtgatgcatgaagccctgcacaatcattacactcagaagagcctgtccctgtctcccggcaaa

SEQ ID NO: 281 - protein, 120 aa, synthetic construct [sequence omitted]

SEQ ID NO: 282 - DNA, 360 bp, synthetic construct; identical to SEQ ID NO: 4
  misc_feature 1..360: note = Description of Artificial Sequence: Synthetic polynucleotide
  source 1..360: mol_type = other DNA

SEQ ID NO: 283 - protein, 8 aa, synthetic construct
  REGION 1..8: note = Description of Artificial Sequence: Synthetic peptide
GFNIKDTY

SEQ ID NO: 284 - DNA, 24 bp, synthetic construct
  misc_feature 1..24: note = Description of Artificial Sequence: Synthetic oligonucleotide
  source 1..24: mol_type = other DNA
ggattcaacatcaaggacacctac

SEQ ID NO: 285 - protein, 13 aa, synthetic construct
  REGION 1..13: note = Description of Artificial Sequence: Synthetic peptide
SRWGGDGFYAMDY

SEQ ID NO: 286 - DNA, 39 bp, synthetic construct; identical to SEQ ID NO: 8
  misc_feature 1..39: note = Description of Artificial Sequence: Synthetic oligonucleotide
  source 1..39: mol_type = other DNA

SEQ ID NO: 287 - protein, 8 aa, synthetic construct
  REGION 1..8: note = Description of Artificial Sequence: Synthetic peptide
IYPTNGYT

SEQ ID NO: 288 - DNA, 24 bp, synthetic construct
  misc_feature 1..24: note = Description of Artificial Sequence: Synthetic oligonucleotide
  source 1..24: mol_type = other DNA
atctatcccactaatggatacacc

SEQ ID NO: 289 - protein, 98 aa, synthetic construct; identical to SEQ ID NO: 11
  REGION 1..98: note = Description of Artificial Sequence: Synthetic polypeptide

SEQ ID NO: 290 - DNA, 294 bp, synthetic construct; identical to SEQ ID NO: 12
  misc_feature 1..294: note = Description of Artificial Sequence: Synthetic polynucleotide
  source 1..294: mol_type = other DNA

SEQ ID NO: 291 - protein, 110 aa, synthetic construct; identical to SEQ ID NO: 13
  REGION 1..110: note = Description of Artificial Sequence: Synthetic polypeptide

SEQ ID NO: 292 - DNA, 330 bp, synthetic construct; identical to SEQ ID NO: 14
  misc_feature 1..330: note = Description of Artificial Sequence: Synthetic polynucleotide
  source 1..330: mol_type = other DNA

SEQ ID NO: 293 - protein, 106 aa, synthetic construct; identical to SEQ ID NO: 31
  REGION 1..106: note = Description of Artificial Sequence: Synthetic polypeptide

SEQ ID NO: 294 - DNA, 318 bp, synthetic construct
  misc_feature 1..318: note = Description of Artificial Sequence: Synthetic polynucleotide
  source 1..318: mol_type = other DNA
ggccagccaagggagccccaggtgtacgtgctgccacccagcagagacgaactgaccaagaaccaggtgtccctgctgtgtctggtgaaaggcttctatcctagtgatattgctgtggagtgggaatcaaatggacagccagagaacaattacctgacctggcctccagtgctggacagcgatggcagcttcttcctgtattccaagctgacagtggataaatctcgatggcagcaggggaacgtgtttagttgttcagtgatgcatgaagccctgcacaatcattacactcagaagagcctgtccctgtctcccggc

SEQ ID NO: 295 - protein, 480 aa, synthetic construct
  REGION 1..480: note = Description of Artificial Sequence: Synthetic polypeptide
DIQMTQSPSSLSASVGDRVTITCRASQDVNTAVAWYQQKPGKAPKLLIYSASFLYSGVPSRFSGSRSGTDFTLTISSLQPEDFATYYCQQHYTTPPTFGQGTKVEIKGGSGGGSGGGSGGGSGGGSGEVQLVESGGGLVQPGGSLRLSCAASGFNIKDTYIHWVRQAPGKGLEWVARIYPTNGYTRYADSVKGRFTISADTSKNTAYLQMNSLRAEDTAVYYCSRWGGDGFYAMDYWGQGTLVTVSSAAEPKSSDKTHTCPPCPAPELLGGPSVFLFPPKPKDTLMISRTPEVTCVVVDVSHEDPEVKFNWYVDGVEVHNAKTKPREEQYNSTYRVVSVLTVLHQDWLNGKEYKCKVSNKALPAPIEKTISKAKGQPREPQVYVLPPSRDELTKNQVSLLCLVKGFYPSDIAVEWESNGQPENNYLTWPPVLDSDGSFFLYSKLTVDKSRWQQGNVFSCSVMHEALHNHYTQKSLSLSPG

SEQ ID NO: 296 - DNA, 1440 bp, synthetic construct
  misc_feature 1..1440: note = Description of Artificial Sequence: Synthetic polynucleotide
  source 1..1440: mol_type = other DNA
gacattcagatgacacagagccccagctccctgagtgcttcagtcggcgacagggtgactatcacctgccgcgcatcccaggatgtcaacaccgctgtggcatggtaccagcagaagcctggaaaagccccaaagctgctgatctacagcgcttccttcctgtattctggcgtgccaagtcggttttctggaagtagatcaggcactgacttcacactgactatctctagtctgcagcccgaagattttgccacctactattgccagcagcactataccacaccccctacattcggacagggcactaaagtggagattaagggcgggtcaggcggagggagcggaggagggtccggaggagggtctggaggagggagtggagaggtccagctggtggaatctggaggaggactggtgcagcctggaggctcactgcgactgagctgtgccgcttccggctttaacatcaaagacacatacattcattgggtcaggcaggcaccagggaagggactggaatgggtggcccgcatctatcccacaaatgggtacactcgatatgccgacagcgtgaaaggacggtttaccatttctgctgataccagtaagaacacagcatacctgcagatgaacagcctgcgcgcagaggatacagccgtgtactattgcagtcgatgggggggagacggcttctacgccatggattattggggccaggggactctggtcaccgtgtcaagcgcagccgaacctaaatcctctgacaagacccacacatgcccaccctgtcctgctccagagctgctgggaggaccatccgtgttcctgtttcctccaaagcctaaagatacactgatgattagccgcactcccgaagtcacctgtgtggtcgtggacgtgtcccacgaggaccccgaagtcaagttcaactggtacgtggacggcgtcgaggtgcataatgccaagactaaaccaagagaggaacagtacaattcaacctatagggtcgtgagcgtcctgacagtgctgcatcaggattggctgaacggcaaggagtataagtgcaaagtgtctaacaaggccctgcccgctcctatcgagaagactattagcaaggcaaaagggcagccacgggaaccccaggtctacgtgctgccccctagcagagacgagctgaccaaaaaccaggtctccctgctgtgtctggtgaagggcttttatcctagtgatatcgctgtggagtgggaatcaaatgggcagccagaaaacaattacctgacatggccacccgtgctggacagcgatgggtccttctttctgtattccaaactgactgtggacaagtctagatggcagcagggaaacgtcttcagctgttccgtgatgcacgaggccctgcacaatcattacacccagaagtctctgagtctgtcacccggc

SEQ ID NO: 297 - protein, 107 aa, synthetic construct [sequence omitted]

SEQ ID NO: 298 - DNA, 321 bp, synthetic construct
  misc_feature 1..321: note = Description of Artificial Sequence: Synthetic polynucleotide
  source 1..321: mol_type = other DNA
gacattcagatgacacagagccccagctccctgagtgcttcagtcggcgacagggtgactatcacctgccgcgcatcccaggatgtcaacaccgctgtggcatggtaccagcagaagcctggaaaagccccaaagctgctgatctacagcgcttccttcctgtattctggcgtgccaagtcggttttctggaagtagatcaggcactgacttcacactgactatctctagtctgcagcccgaagattttgccacctactattgccagcagcactataccacaccccctacattcggacagggcactaaagtggagattaag

SEQ ID NO: 299 - protein, 6 aa, synthetic construct
  REGION 1..6: note = Description of Artificial Sequence: Synthetic peptide
QDVNTA

SEQ ID NO: 300 - DNA, 18 bp, synthetic construct
  misc_feature 1..18: note = Description of Artificial Sequence: Synthetic oligonucleotide
  source 1..18: mol_type = other DNA
caggatgtcaacaccgct

SEQ ID NO: 301 - protein, 9 aa, synthetic construct
  REGION 1..9: note = Description of Artificial Sequence: Synthetic peptide
QQHYTTPPT

SEQ ID NO: 302 - DNA, 27 bp, synthetic construct
  misc_feature 1..27: note = Description of Artificial Sequence: Synthetic oligonucleotide
  source 1..27: mol_type = other DNA
cagcagcactataccacaccccctaca

SEQ ID NO: 303-304 - skipped (2 entries)

SEQ ID NO: 305 - protein, 120 aa, synthetic construct [sequence omitted]

SEQ ID NO: 306 - DNA, 360 bp, synthetic construct
  misc_feature 1..360: note = Description of Artificial Sequence: Synthetic polynucleotide
  source 1..360: mol_type = other DNA
gaggtccagctggtggaatctggaggaggactggtgcagcctggaggctcactgcgactgagctgtgccgcttccggctttaacatcaaagacacatacattcattgggtcaggcaggcaccagggaagggactggaatgggtggcccgcatctatcccacaaatgggtacactcgatatgccgacagcgtgaaaggacggtttaccatttctgctgataccagtaagaacacagcatacctgcagatgaacagcctgcgcgcagaggatacagccgtgtactattgcagtcgatgggggggagacggcttctacgccatggattattggggccaggggactctggtcaccgtgtcaagc

SEQ ID NO: 307 - protein, 8 aa, synthetic construct
  REGION 1..8: note = Description of Artificial Sequence: Synthetic peptide
GFNIKDTY

SEQ ID NO: 308 - DNA, 24 bp, synthetic construct
  misc_feature 1..24: note = Description of Artificial Sequence: Synthetic oligonucleotide
  source 1..24: mol_type = other DNA
ggctttaacatcaaagacacatac

SEQ ID NO: 309 - protein, 13 aa, synthetic construct
  REGION 1..13: note = Description of Artificial Sequence: Synthetic peptide
SRWGGDGFYAMDY

SEQ ID NO: 310 - DNA, 39 bp, synthetic construct
  misc_feature 1..39: note = Description of Artificial Sequence: Synthetic oligonucleotide
  source 1..39: mol_type = other DNA
agtcgatgggggggagacggcttctacgccatggattat

SEQ ID NO: 311 - protein, 8 aa, synthetic construct
  REGION 1..8: note = Description of Artificial Sequence: Synthetic peptide
IYPTNGYT

SEQ ID NO: 312 - DNA, 24 bp, synthetic construct
  misc_feature 1..24: note = Description of Artificial Sequence: Synthetic oligonucleotide
  source 1..24: mol_type = other DNA
atctatcccacaaatgggtacact

SEQ ID NO: 313 - protein, 110 aa, synthetic construct; identical to SEQ ID NO: 13
  REGION 1..110: note = Description of Artificial Sequence: Synthetic polypeptide

SEQ ID NO: 314 - DNA, 330 bp, synthetic construct
  misc_feature 1..330: note = Description of Artificial Sequence: Synthetic polynucleotide
  source 1..330: mol_type = other DNA
gctccagagctgctgggaggaccatccgtgttcctgtttcctccaaagcctaaagatacactgatgattagccgcactcccgaagtcacctgtgtggtcgtggacgtgtcccacgaggaccccgaagtcaagttcaactggtacgtggacggcgtcgaggtgcataatgccaagactaaaccaagagaggaacagtacaattcaacctatagggtcgtgagcgtcctgacagtgctgcatcaggattggctgaacggcaaggagtataagtgcaaagtgtctaacaaggccctgcccgctcctatcgagaagactattagcaaggcaaaa

SEQ ID NO: 315 - protein, 106 aa, synthetic construct; identical to SEQ ID NO: 31
  REGION 1..106: note = Description of Artificial Sequence: Synthetic polypeptide

SEQ ID NO: 316 - DNA, 318 bp, synthetic construct
  misc_feature 1..318: note = Description of Artificial Sequence: Synthetic polynucleotide
  source 1..318: mol_type = other DNA
gggcagccacgggaaccccaggtctacgtgctgccccctagcagagacgagctgaccaaaaaccaggtctccctgctgtgtctggtgaagggcttttatcctagtgatatcgctgtggagtgggaatcaaatgggcagccagaaaacaattacctgacatggccacccgtgctggacagcgatgggtccttctttctgtattccaaactgactgtggacaagtctagatggcagcagggaaacgtcttcagctgttccgtgatgcacgaggccctgcacaatcattacacccagaagtctctgagtctgtcacccggc

SEQ ID NO: 317 - protein, 214 aa, synthetic construct; identical to SEQ ID NO: 191
  REGION 1..214: note = Description of Artificial Sequence: Synthetic polypeptide

SEQ ID NO: 318 - DNA, 642 bp, synthetic construct
  misc_feature 1..642: note = Description of Artificial Sequence: Synthetic polynucleotide
  source 1..642: mol_type = other DNA
gacatccagatgacccagtctccatcctccctgtctgcatctgtaggagacagagtcaccatcacttgccgggcaagtcaggacgttaacaccgctgtagcttggtatcagcagaaaccagggaaagcccctaagctcctgatctattctgcatcctttttgtacagtggggtcccatcaaggttcagtggcagtcgatctgggacagatttcactctcaccatcagcagtctgcaacctgaagattttgcaacttactactgtcaacagcattacactaccccacccactttcggccaagggaccaaagtggagatcaaacgaactgtggctgcaccatctgtcttcatcttcccgccatctgatgagcagttgaaatctggaactgcctctgttgtgtgcctgctgaataacttctatcccagagaggccaaagtacagtggaaggtggataacgccctccaatcgggtaactcccaagagagtgtcacagagcaggacagcaaggacagcacctacagcctcagcagcaccctgacgctgagcaaagcagactacgagaaacacaaagtctacgcctgcgaagtcacccatcagggcctgagctcgcccgtcacaaagagcttcaacaggggagagtgt

SEQ ID NO: 319 - protein, 107 aa, synthetic construct [sequence omitted]

SEQ ID NO: 320 - DNA, 321 bp, synthetic construct; identical to SEQ ID NO: 150
  misc_feature 1..321: note = Description of Artificial Sequence: Synthetic polynucleotide
  source 1..321: mol_type = other DNA

SEQ ID NO: 321 - protein, 6 aa, synthetic construct
  REGION 1..6: note = Description of Artificial Sequence: Synthetic peptide
QDVNTA

SEQ ID NO: 322 - DNA, 18 bp, synthetic construct
  misc_feature 1..18: note = Description of Artificial Sequence: Synthetic oligonucleotide
  source 1..18: mol_type = other DNA
caggacgttaacaccgct

SEQ ID NO: 323 - protein, 9 aa, synthetic construct
  REGION 1..9: note = Description of Artificial Sequence: Synthetic peptide
QQHYTTPPT

SEQ ID NO: 324 - DNA, 27 bp, synthetic construct
  misc_feature 1..27: note = Description of Artificial Sequence: Synthetic oligonucleotide
  source 1..27: mol_type = other DNA
caacagcattacactaccccacccact

SEQ ID NO: 325-326 - skipped (2 entries)

SEQ ID NO: 327 - protein, 107 aa, synthetic construct [sequence omitted]

SEQ ID NO: 328 - DNA, 321 bp, synthetic construct
  misc_feature 1..321: note = Description of Artificial Sequence: Synthetic polynucleotide
  source 1..321: mol_type = other DNA
cgaactgtggctgcaccatctgtcttcatcttcccgccatctgatgagcagttgaaatctggaactgcctctgttgtgtgcctgctgaataacttctatcccagagaggccaaagtacagtggaaggtggataacgccctccaatcgggtaactcccaagagagtgtcacagagcaggacagcaaggacagcacctacagcctcagcagcaccctgacgctgagcaaagcagactacgagaaacacaaagtctacgcctgcgaagtcacccatcagggcctgagctcgcccgtcacaaagagcttcaacaggggagagtgt

SEQ ID NO: 329 - protein, 231 aa, synthetic construct
  REGION 1..231: note = Description of Artificial Sequence: Synthetic polypeptide
EPKSSDKTHTCPPCPAPELLGGPSVFLFPPKPKDTLMISRTPEVTCVVVDVSHEDPEVKFNWYVDGVEVHNAKTKPREEQYNSTYRVVSVLTVLHQDWLNGKEYKCKVSNKALPAPIEKTISKAKGQPREPQVYVLPPSRDELTKNQVSLLCLVKGFYPSDIAVEWESNGQPENNYLTWPPVLDSDGSFFLYSKLTVDKSRWQQGNVFSCSVMHEALHNHYTQKSLSLSPG

SEQ ID NO: 330 - DNA, 693 bp, synthetic construct
  misc_feature 1..693: note = Description of Artificial Sequence: Synthetic polynucleotide
  source 1..693: mol_type = other DNA
gaacctaaatccagcgacaagacccacacatgccccccttgtccagctccagaactgctgggaggaccaagcgtgttcctgtttccacccaagcccaaagatacactgatgatcagccgaactcccgaggtcacctgcgtggtcgtggacgtgtcccacgaggaccccgaagtcaagttcaactggtacgtggacggcgtcgaagtgcataatgcaaagactaaaccacgggaggaacagtacaactctacatatagagtcgtgagtgtcctgactgtgctgcatcaggattggctgaacggcaaagagtataagtgcaaagtgtctaataaggccctgcctgctccaatcgagaaaactattagtaaggcaaaagggcagcccagggaacctcaggtctacgtgctgcctccaagtcgcgacgagctgaccaagaaccaggtctcactgctgtgtctggtgaaaggattctatccttccgatattgccgtggagtgggaatctaatggccagccagagaacaattacctgacctggccccctgtgctggacagcgatgggtccttctttctgtattcaaagctgacagtggacaaaagcagatggcagcagggaaacgtctttagctgttccgtgatgcacgaagccctgcacaatcattacacccagaagtctctgagtctgtcacctggc

SEQ ID NO: 331 - protein, 110 aa, synthetic construct; identical to SEQ ID NO: 13
  REGION 1..110: note = Description of Artificial Sequence: Synthetic polypeptide

SEQ ID NO: 332 - DNA, 330 bp, synthetic construct; identical to SEQ ID NO: 254
  misc_feature 1..330: note = Description of Artificial Sequence: Synthetic polynucleotide
  source 1..330: mol_type = other DNA

SEQ ID NO: 333 - protein, 106 aa, synthetic construct; identical to SEQ ID NO: 31
  REGION 1..106: note = Description of Artificial Sequence: Synthetic polypeptide

SEQ ID NO: 334 - DNA, 318 bp, synthetic construct; identical to SEQ ID NO: 256
  misc_feature 1..318: note = Description of Artificial Sequence: Synthetic polynucleotide
  source 1..318: mol_type = other DNA

SEQ ID NO: 335 - protein, 8 aa, synthetic construct
  REGION 1..8: note = Description of Artificial Sequence: Synthetic peptide
VNPNSGGS

SEQ ID NO: 336 - protein, 12 aa, synthetic construct
  REGION 1..12: note = Description of Artificial Sequence: Synthetic peptide
ARNLGPSFYFDY

SEQ ID NO: 337 - protein, 8 aa, synthetic construct
  REGION 1..8: note = Description of Artificial Sequence: Synthetic peptide
GFTFTDYT

SEQ ID NO: 338 - skipped

SEQ ID NO: 339 - protein, 9 aa, synthetic construct
  REGION 1..9: note = Description of Artificial Sequence: Synthetic peptide
QQYYIYPYT

SEQ ID NO: 340 - protein, 6 aa, synthetic construct
  REGION 1..6: note = Description of Artificial Sequence: Synthetic peptide
QDVSIG

SEQ ID NO: 341 - protein, 8 aa, synthetic construct
  REGION 1..8: note = Description of Artificial Sequence: Synthetic peptide
IYPTNGYT

SEQ ID NO: 342 - protein, 13 aa, synthetic construct
  REGION 1..13: note = Description of Artificial Sequence: Synthetic peptide
SRWGGDGFYAMDY

SEQ ID NO: 343 - protein, 8 aa, synthetic construct
  REGION 1..8: note = Description of Artificial Sequence: Synthetic peptide
GFNIKDTY

SEQ ID NO: 344 - skipped

SEQ ID NO: 345 - protein, 9 aa, synthetic construct
  REGION 1..9: note = Description of Artificial Sequence: Synthetic peptide
QQHYTTPPT

SEQ ID NO: 346 - protein, 6 aa, synthetic construct
  REGION 1..6: note = Description of Artificial Sequence: Synthetic peptide
QDVNTA

SEQ ID NO: 347 - protein, 9 aa, synthetic construct
  REGION 1..9: note = Description of Artificial Sequence: Synthetic peptide
QQYYIYPAT

SEQ ID NO: 348 - protein, 8 aa, synthetic construct
  REGION 1..8: note = Description of Artificial Sequence: Synthetic peptide
GFTFADYT

SEQ ID NO: 349 - protein, 607 aa, Homo sapiens
TQVCTGTDMKLRLPASPETHLDMLRHLYQGCQVVQGNLELTYLPTNASLSFLQDIQEVQGYVLIAHNQVRQVPLQRLRIVRGTQLFEDNYALAVLDNGDPLNNTTPVTGASPGGLRELQLRSLTEILKGGVLIQRNPQLCYQDTILWKDIFHKNNQLALTLIDTNRSRACHPCSPMCKGSRCWGESSEDCQSLTRTVCAGGCARCKGPLPTDCCHEQCAAGCTGPKHSDCLACLHFNHSGICELHCPALVTYNTDTFESMPNPEGRYTFGASCVTACPYNYLSTDVGSCTLVCPLHNQEVTAEDGTQRCEKCSKPCARVCYGLGMEHLREVRAVTSANIQEFAGCKKIFGSLAFLPESFDGDPASNTAPLQPEQLQVFETLEEITGYLYISAWPDSLPDLSVFQNLQVIRGRILHNGAYSLTLQGLGISWLGLRSLRELGSGLALIHHNTHLCFVHTVPWDQLFRNPHQALLHTANRPEDECVGEGLACHQLCARGHCWGPGPTQCVNCSQFLRGQECVEECRVLQGLPREYVNARHCLPCHPECQPQNGSVTCFGPEADQCVACAHYKDPPFCVARCPSGVKPDLSYMPIWKFPDEEGACQPCPIN

SEQ ID NO: 350 - protein, 217 aa, Homo sapiens
APELLGGPSVFLFPPKPKDTLMISRTPEVTCVVVDVSHEDPEVKFNWYVDGVEVHNAKTKPREEQYNSTYRVVSVLTVLHQDWLNGKEYKCKVSNKALPAPIEKTISKAKGQPREPQVYTLPPSRDELTKNQVSLTCLVKGFYPSDIAVEWESNGQPENNYKTTPPVLDSDGSFFLYSKLTVDKSRWQQGNVFSCSVMHEALHNHYTQKSLSLSPGK